European Patent Specification EP 3 722 306 B1, published November 6, 2024. Title: MODIFIED CULLIN1 GENE. Applicant: Rijk Zwaan Zaadteelt en Zaadhandel B.V. The sequence listing filed with the application follows.

SEQUENCE LISTING (69 sequences)

SEQ ID NO: 1 - DNA, 2235 bp, Cucumis sativus
  source 1..2235: /organism="Cucumis sativus" /mol_type="unassigned DNA"
atgacaatgggcgagcggaagactattgacttggagcagggatgggagtttatgcagaagggtatcacaaagttgaagaacattctcgagggcttgcctgagcctcagttcagctccgaggactacatgatgctttacactaccatatataacatgtgcacccaaaagccgccgcatgattactcccagcagctgtatgataaatatcgtgaatcttttgaagagtacatcacttctatggtcttaccatccttgagggagaagcacgatgagttcatgttgagagaactagtaaaaaggtggacaaaccataaagtcatggtgaggtggctttctcgcttcttccactatcttgatcggtacttcatcgctcgaaggtcacttccacctctaaatgaagttggcctcacatgcttccgcgaattggtgtacaaagagctaaatagtaaagtgagggatgcagtaatttcattgattgatcaagaacgtgaaggagaacagattgacagagctctactgaagaatgtactagatatatttgtggaaattggtatggggcaaatggattactatgaaaatgactttgaagctgccatgcttaaagatactgctgcttattactctaggaaggcttccaattggatcctagaagattcttgtcccgattatatgcttaaagcagaggagtgcttgaaacgagaaaaggatagggtttcccactatttgcactctagtagcgagccaaagttgttggagaaagttcaacatgaactattatctgtttatgctactcaactgctggaaaaagagcattcaggatgccatgcattgcttagagatgacaaggtggaagatttgtcaaggatgttccgtctattctccaaaataccgaagggactggatccagtttccaacatatttaagcagcatgtaactgctgaaggaacagcactggtcaaacaggcagaagatgctgcaagtaacaagaaggctgagaaaaaggacatagttggtctgcaggaacaggtttttgtaagaaaagtgattgagcttcacgacaagtacttggcttatgtgaatgattgtttccaaaaccacacacttttccataaggctctcaaggaagcttttgaagtattttgcaataagggtgttgctggaagttctagtgcagaattgcttgctaccttttgtgataacatccttaagaaaggtgggagtgagaagttgagtgatgaagcaatcgaggagacacttgagaaggttgtgaagttgttggcatacatttgcgacaaagatctgtttgctgaattctatagaaaaaaacttgcccgaaggcttctctttgacaagagcgcgaacgatgaccacgagagaagtatattgaccaaattgaagcaacaatgtggtggtcagttcacttctaagatggagggaatggttactgatttgactttggcaagggagaaccaaactagttttgaggagtatctgagcaataatccacaagcgagtcctggcatcgacctgactgttactgttttaactactggattttggccaagctacaagtcttttgacctcaacctgccggcagagatggtaaagtgtgttgaagttttcagagagttttatcaaacaaaaaccaagcatcgaaaacttacatggatttactcattgggtacttgtaacatcagtggaaaatttgaaccgaaaacgatggagctgattgtgacaacttatcaggcttctgccctgttgctattcaattcttcggatagactaagttactcggaaatcatgacacaattaaatttgagtgacgatgatgtagttagactactccactcgttgtcatgtgccaagtataaaattcttaataaggaaccaaatacgaaaaccatctctccgaacgatcattttgagttcaatgcaaaattctccgacaaaatgaggagaataaagatccctcttccgcctgtggatgagaaaaagaaagtcattgaagatgttgacaaggatcgaaggtatgctattgacgcctcaatcgtgcgtatcatgaagagtcggaaagttcttggtcatcagcaactagtgatggagtgcgtcgagcaattgggccgtatgttcaagcccgatttcaaggcgataaagaagagaattgaagacctgatcactcgggattatctagagagagacaaagacaacccccacttgtttaggtacttggcttga

SEQ ID NO: 2 - DNA, 2235 bp, Cucumis melo
  source 1..2235: /organism="Cucumis melo" /mol_type="unassigned DNA"
atgacaatgggcgagcggaagactattgacttggaacagggatgggagtttatgcagaagggtatcacaaagttgaagaacattcttgagggcttgcctgagccccagttcagctccgaggactacatgatgctttacactaccatatataacatgtgcacccaaaagccgccgcatgattactcccagcagctgtatgataaatatcgtgaatcttttgaagagtacatcacttctatggtcttaccatccttgagggagaagcatgacgagttcatgttgagagaactagtcaaaaggtggacaaaccataaagtcatggtgaggtggctttctcgcttcttccactatcttgatcggtacttcatcgctcgaaggtcacttccacctctaaatgaagttggcctcacatgcttccgcgaattggtgtacaaagagctaaacagtaaagtgagggatgcagtaatctcattgattgatcaagaacgtgaaggagaacagattgacagagctctactgaagaatgtattagatatatttgtggaaattggtatggggcaaatggattactatgaaaatgactttgaagctgccatgcttaaagatactgctgcttattactctaggaaggcttccaattggatcctagaagattcttgtcccgattatatgctaaaagcagaggagtgcttgaagcgagaaaaggatagggtttcccactatttgcactctagtagcgagccaaagttgttggagaaagttcaacacgaactgttatctgtgtatgctactcaactgctggaaaaagagcattcaggatgccatgcattgcttagagatgacaaggtggaagatttgtcaaggatgttccgtctcttctccaaaataccgaagggattggacccagtttccaacatatttaagcagcatgtaactgctgaaggaacagcactggtcaaacaggcagaagatgctgcaagtaacaagaaggccgagaaaaaggacatagttggtctgcaggaacaggtttttgtaagaaaagtgattgagcttcacgacaagtacttggcttatgtgaatgattgtttccaaaaccacacacttttccataaggctctcaaggaagcttttgaagtcttttgcaataagggtgttgctggaagttctagtgcagaattgcttgctaccttctgcgataacatccttaagaaaggtgggagtgagaagttgagtgatgaagcaatcgaagagacacttgagaaggttgtgaagttgttggcatacatctgcgacaaagatctgtttgctgaattctatagaaaaaaacttgcccgaaggcttctctttgataagagcgccaacgatgaccacgagagaagtatattgaccaaattgaagcaacaatgtggtggtcagttcacttctaagatggagggaatggttactgatttgactttggcaagggagaaccaaactagtttcgaagagtatctgagcaataatccacaagctagtcctggaatcgacctaactgttactgttttgactactggattttggccaagctacaagtcttttgacctcaacctgccggcggagatggtaaagtgtgttgaagttttcagagagttttatcaaacaaaaaccaagcatagaaaacttacatggatttactcattgggtacttgtaacatcagtggaaaatttgaaccgaagacgatggagctgattgtgacaacatatcaggcttctgccctgttgctattcaattcttcggacagactaagttactccgaaatcatgacacaattaaatttgagtgatgatgatgttgttagactgctccactcattgtcgtgtgccaagtataaaattcttaataaggagccaaatacgaaaaccatctcaccgaacgatcattttgagttcaatgcaaaattctccgacaaaatgaggagaataaagatccctcttccgcctgtggatgagaaaaagaaagtcattgaagatgttgacaaggatcgaaggtatgctattgacgcctcaatcgtgcgtatcatgaagagtcgaaaagttcttggtcatcagcaactagtgatggagtgcgtcgagcaattgggtcgtatgttcaagcccgatttcaaggcgataaagaagagaattgaagacctgatcactcgggactatctagagagagacaaagacaacccccacttgtttaggtacttggcttga

SEQ ID NO: 3 - DNA, 2235 bp, Cucurbita pepo
  source 1..2235: /organism="Cucurbita pepo" /mol_type="unassigned DNA"
atgacaatgggtgagcggaagactattgacttggagcaaggatgggagtttatgcagaagggaatcacaaaattgaagaacattctggaaggattgcctgagccacagttcagctccgaggactacatgatgctttacactacaatatataacatgtgtacccagaagccaccgcatgattactcccagcagctgtatgataaataccgcgaatcgtttgaggagtacatcagttctatggttttaccatccttgagggagaagcatgacgaatttatgttgagagaactggtcaaaaggtggaccaaccataaagtcatggtgaggtggctttctcgcttcttccactatcttgatcgatacttcattgctcgaaggtcacttccacctctcaatgaagttggcctcacttgcttccgtgaattggtgtacaaagagctaaacagtaaagtgagggatgcagtaatttcattgatcgatcaagaacgtgaaggagagcagattgacagagctctgttgaagaacgtgttggatatatttgtggagattgggatggggcaaatggattattatgaaaatgactttgaagctgccatgcttaaagatactgctgcttactactctaggaaggcatcaaattggatcttagaagattcttgtcctgattatatgctaaaagcagaggagtgcttgagacgagaaaaggaccgagtttctcactatctgcactctagtagcgagccaaagttattggagaaagttcaacatgaactattgtctgtttatgctactcaactgctggagaaagagcattcaggatgccatgcattgcttagagatgacaaggtggaagatttgtcaaggatgttccgtctcttctccaaaatacccaagggattggacccagtttccaacatatttaagcagcatgtcactgctgaaggaacagcattagtcaaacaggcagaagacgctgcaagtaacaagaaggccgagaaaaaggacatcgttggtctgcaagaacaggtttttgttagaaaagtgattgagcttcacgacaagtacttggcatatgtgaatgattgtttccaaaaccacacactttttcacaaggctctcaaggaagcttttgaagtcttttgcaataagggtgttgctggaagttctagtgcagaattacttgctaccttttgtgataacatccttaagaaaggtgggagtgagaagttgagtgatgaagcaattgaggaaacactcgagaaggtcgtgaaattgctggcgtatatctgcgacaaagatctgtttgctgaattctatagaaaaaaactcgcccgaaggcttctcttcgacaagagtgcgaatgatgaccacgagagaagtatactgacgaaattgaagcaacaatgtggtggtcagtttacctctaagatggagggaatggtcacggatttgacactggcaagggagaaccaaactagttttgaggaatatctgagcaataatccacaagctagtcctggaatcgacttgaccgttaccgttttgaccactggtttttggccaagctacaagtcttttgacctcaacctgccggcggagatggtaaagtgtgttgaagttttcagggaattttatcaaacaaaaaccaagcacagaaaacttacgtggatttactcgttgggtacctgtaacatcagcggaaaattcgaaccgaaaacgatggagctgatcgtgacaacctatcaggcttctgccctgctgcttttcaattcctcggataaactaagttactccgagatcatgactcaattaaacttgagtgacgatgatgttgttagactgctccactcgttgtcgtgtgcgaagtataaaattcttaacaaggagccaaatacgaaaaccatctctccgaacgatcattttgagttcaacgcaaaattctccgacaaaatgaggagaataaagatccctcttccgcctgtggatgagaaaaagaaagtaatagaagatgttgacaaggatcgaagatatgctatcgatgcctcgatcgtgcgtatcatgaagagtaggaaagttctgggtcaccagcagttagtgatggagtgcgtcgagcaactgggtcgtatgttcaagcctgatttcaaggcgataaagaagagaatcgaagatctgatcactcgtgactatttagagagagacaaagacaacccccacttgtttaggtacttggcttga

SEQ ID NO: 4 - DNA, 2235 bp, citrillus lanatus
  source 1..2235: /organism="citrillus lanatus" /mol_type="unassigned DNA"
atgacaatgggcgagcggaagactattgacttggaacaaggatgggagtttatgcagaagggaatcacaaagttgaagaacattcttgagggcttgcctgagcctcagttcagctccgaggactacatgatgctttataccaccatatacaacatgtgcacacaaaagccgccacatgattactcccagcagctatacgataaataccgtgaatcttttgaggagtatatcacttctatggtcttaccatccttgagggagaagcatgacgagttcatgttgagagaactggtcaaaaggtggacgaaccataaagtcatggtgaggtggctttctcgcttcttccactatcttgaccgatacttcattgctcgaagatcacttccacctctcaacgaagttggcctcacatgcttccgtgaattggtgtacaaagagctaaacagtaaagtgagggatgcagtaatttcattgattgatcaagaacgtgaaggagagcagattgacagagctctactgaagaatgtattagatatatttgtggaaattgggatggggcaaatggattactatgaaaatgactttgaagctgccatgcttaaagatactgctgcttattactctaggaaggcttccaattggatcctagaagattcttgtcccgattatatgctaaaagcagaggagtgcttgaaacgagaaaaggatagagtttctcactatttgcactctagtagcgagccaaagttattagagaaagttcaacatgaactgttatctgtgtatgctactcaactgctggaaaaagagcattcaggatgccatgcattgcttagagatgacaaggtggaagatttgtcaaggatgttccgcctcttctccaaaatacccaagggattggacccagtttccaacatatttaagcagcatgtcactgctgaaggaacagcattggtcaaacaggcagaagatgctgcaagtaacaagaaggccgagaaaaaggacatagttggtctgcaggaacaggtttttgtaagaaaagtgattgagcttcacgacaagtacttggcttacgtgaatgattgtttccaaaaccacacactttttcacaaggctctcaaggaagcttttgaagtcttttgcaataagggtgttgctggaagttctagtgcagaattacttgctaccttttgtgataacatccttaagaaaggtgggagcgagaagttgagtgatgaagcaattgaggagacacttgagaaggtcgtgaagttgctggcatacatctgcgacaaagatctgtttgctgaattctatagaaaaaaacttgcccgaaggcttctctttgacaagagtgccaacgatgaccatgagagaagtatattgaccaaattgaagcaacaatgtggtggccagttcacctctaagatggaggggatggtcactgatttgactttggcaagggagaaccaaactagtttcgaggagtatctgagcaataatccacaagctagtcctggaatcgacttgactgtcactgttttgactactggcttttggccaagctacaagtcttttgacctcaacctgccggcagagatggtaaagtgtgttgaagttttcagagagttctatcaaacaaaaacaaagcatagaaaacttacatggatttactcattgggtacctgtaacatcagcggaaaatttgaaccgaaaacgatggagctgattgtaacaacttatcaggcttctgccctgctgctattcaattcctcagatagattaagttattccgagatcatgacacaattaaatttgagtgacgatgatgttgttagactgctccactcattgtcatgtgccaagtataaaattcttaataaggagccgaacacgaaaaccatctctccgaatgatcattttgagttcaatgcaaaattctccgacaaaatgaggagaataaagatccctcttccgcctgtggatgagaaaaagaaagtcattgaagatgttgacaaggatcgaaggtatgctattgatgcctcaatcgtgcgtatcatgaagagtcggaaagttctgggtcatcagcagctagtgatggagtgcgtcgagcaattgggtcgtatgttcaagcccgacttcaaagcgataaagaagagaatcgaagatctgatcactcgggactatttagagagagacaaagacaacccccacttgtttaggtacttggcttga

SEQ ID NO: 5 - DNA, 2229 bp, Solanum melongena
  source 1..2229: /organism="Solanum melongena" /mol_type="unassigned DNA"
atgaaccaacgcagcacaatcgatctggaacatggatgggatttcatgcaaaagggcatcacaaagctgaagaacattctagaagggctgcctgagcctcagttcagctcagaggactatatgatgctgtatacgacaatttacaacatgtgtactcagaagcccccacatgattattctcaacagctgtatgacaaatatcgtgaagcttttgaagaatatatcacaacgacggtattaccttctttgagagaaaaacatgacgagttcatgttgcgagagttggtaaaaaggtggtcaaaccataaggtcatggttagatggttatcgcgattcttccattatcttgaccgttatttcattgctcggagatcactgccagggcttaatgaagttggactaacttgcttccgcgatctggtctaccaagagttgaatggaaaagtcagggatgctgttatatctctgattgatcaagagcgtgagggagagcaaattgacagagctctactgaagaatgtgctagatatatttgttgaaattggaatggggtcaatggattattatgagaatgattttgaagctgcaatgctcaaggacactgcggcttattattctcgcaaagcttctaactggatcctcgaagattcatgtccagattatatgctgaaagctgaggagtgcttgaaacgggagaaggatagggtctcccattatctccattctagcagtgagacaaagttgcttgagaaagtgcaacatgagttgttatctgtgtatgccaatcaacttcttgagaaggagcactctggatgccatgcattacttagagatgataaggtcgatgatttatcaaggatgtatagactcttttctaagattcctcgaggcttagagcctgtggctaatatatttaagcagcatgttactgctgaaggtacagctttggtgaaacaggctgaagatgctgctagcaacaaaaaggcagagaagagagatgtggttggtttgcaggaacaggtttttgttcggaaagtgattgagcttcatgataaatatttggcgtatgtgaataactgtttccaaaaccacacactttttcacaaggcacttaaagaagctttcgaacttttctgcaacaagggtgttgctggtagctcaaatgctgaacttcttgccacattctgcgacaacattctcaaaaaaggcgggagtgaaaaattgagtgatgaagccattgaagagacgctggagaaggtggtaaagctgctggcttatattagtgataaggacttgtttgcagaattctataggaaaaagctcgcccggcggttgttatttgataagagtgccaatgatgaacatgagagaagtatcctaacaaagttgaagcagcagtgtggaggtcagttcacatcaaagatggagggaatggtcacagatttgacattggcaagggaaaatcaagccagctttgaggagtatttgagcaataatccaacagcaaatccaggaattgacttgacggtgactgtcttgactactggcttctggcctagctacaagtcttttgatctcaacctcccagcagaaatggttaggtgtgttgaagtattcaaggagttttatcaaacaaaaacgaagcacaggaaacttacatggatatactctttgggaacttgcaacataaatggaaaatttgaggcaaagactattgagctcgttgtcactacttatcaggcttctgctctgcttctctttaatgcatcagatagattgagttatcaggaaatcatgacgcaattaaacctatcagatgatgatgttgttcggcttcttcattccctttcatgtgcgaaatacaagattctcaacaaggagccaagcaccaaaacaatttctccgactgatgtctttgagttcaactcaaagttcactgacaaaatgaggaggatcaagatacctctcccaccagttgatgaaaagaaaaaggtaattgaagacgttgacaaggataggcggtatgctatagatgcctcaattgtgcgtattatgaagagtcgtaaagtattgggctaccagcaactggtcatggagtgcgttgagcagttgggacgcatgttcaagcctgatgtcaaagctatcaagaagagaattgaagatctgataactagagattacctagagagggacaaagataacccaaacttgttcaagtacttggcatga

SEQ ID NO: 6 - DNA, 2229 bp, Solanum lycopersicum
  source 1..2229: /organism="Solanum lycopersicum" /mol_type="unassigned DNA"
atgaaccaacgaagcacaatcgatctggaacatggatgggacttcatgcaaaggggcattacaaagctgaagaacattctagaagggctgcctgagcctcaattcagctcagaggactatatgatgctatatacgacaatttacaacatgtgtactcaaaagcccccacatgattattctcaacagctgtatgacaaatatcgtgaagcttttgaagaatatatcacaacaacggtattgccttctttgagagaaaaacatgacgagtttatgttgcgagagttggtaaaaaggtggtcaaatcataaagtcatggtcagatggttgtcaagattcttccattaccttgaccggtatttcattgcccggagatctctgccggggcttaatgaagttggactaacttgcttccgcgatcaggtctaccaagagttgaatggaaaagtcagggatgctgttatatctctgattgatcaagagcgtgagggagagcaaattgacagagctctacttaagaatgtgcttgatatatttgtcgaaattggaatggggttaatggattattatgagaatgattttgaagctgcaatgctcaaggacacagcggcttattattctcgcaaagcttctaattggatcctcgaagattcatgtccggattatatgctgaaagccgaggagtgcttgaaacgggagaaggatagggtctctcattatctccattcaagcagcgagacgaagttgcttgagaaagtgcaacatgagttgttgtctgtgtatgccactcaacttcttgagaaggagcactctggatgccatgcgttactgagagatgataaggttgaagatttatcaaggatgtataggctcttttctaagatttctcgaggcttagaccctgtggccaatatttttaagcagcatgttactgctgaaggtacagctttggtaaaacaggctgaagatgctgctagcaataaaaaggcagagaagagagatgtggttggtttgcaggaacaggtttttgttcggaaagtgattgaacttcatgataaatatttggcttatgtgaataactgtttccaaaaccacacactttttcacaaggcgcttaaagaagcttttgagcttttctgcaacaagggtgttgctggtagctcaagcgctgaacttcttgccaccttctgtgacaacattctcaaaaaaggcgggagtgagaaattgagtgatgaagctattgaagaaacgttggaaaaggtggtaaagctactagcttatattagtgataaggacttgtttgcagaattctataggaaaaagctagcccggcggttgttatttgataagagtgccaatgatgaacatgaaagaagtatcctaacaaagttgaagcagcagtgtggggggcagttcacatcaaagatggagggaatggtcacagatttgacattggcaagggaaaatcaagccagcttcgaggagtatttgagcaataatccaatagcaaatccaggaattgacttgacggtgactgtcttgactactggcttctggcctagctacaagtcttttgatctcaacctcccagcagaaatggttaggtgcgttgaagtatttaaggagttctatcaaacaaaaacaaagcacaggaaacttacgtggatatactctttgggaacttgcaacataaatggaaaatttgagccaaaaactattgagctcgttgtcactacttatcaggcttctgctctgctgctctttaatgcatcagatagattgagttatcaggaaatcatgacgcaattaaacctatcagatgatgatgttgttcggcttcttcattccctttcatgtgcgaagtacaagatactcaacaaggagccaagcaccaaaacaatttctccgactgatgtctttgagttcaactcaaagttcactgacaaaatgaggaggatcaagatacctctccctcctgttgatgagaagaaaaaggtaattgaagacgttgacaaggataggcggtatgctatagatgcttcaattgtgcgtattatgaagagccgtaaagtattgggctaccagcaactagtcatggagtgcgttgagcagttggggcgcatgttcaagcctgatgtcaaagctatcaagaagagaatcgaagatttgataactagagattacctagagagggacaaagataatccaaacctgttcaagtacttggcatga

SEQ ID NO: 7 - DNA, 2229 bp, Capsicum annuum
  source 1..2229: /organism="Capsicum annuum" /mol_type="unassigned DNA"
atgaaccagcgttccacaatcaatctagaacatggatgggacttcatgcaaaggggcattacaaagctgaagaacattctagaagggctgcccgagcctcagttcagctcagaggactatatgatgctgtatacgacaatttacaacatgtgtactcagaagcccccacatgattattctcaacagctgtatgacaaatatcgtgaagcttttgaagaatatatcacaacaacggtattgccttctttgagagaaaaacatgacgagttcatgttgcgagagctggtaaaaaggtggtcaaaccataaggtcatggtcagatggttatcgcgattcttccattatcttgatcgctatttcattgcccggagatctctaccggggcttaatgaagttggactaacttgcttccgagatctggtctaccaagagttgaatggaaaagtcagggatgctgttatatctctgattgatcaagagcgtgagggagagcaaattgacagagctctactgaagaatgtgctagatatatttgttgaaattggaatggggtcgatggattattatgagaatgattttgaagctgcaatgctcaaggacaccgcagcttattattctcgcaaagcttctaactggatacttgaagattcatgtccagattatatgctgaaagccgaggagtgcttgaaacgggagaaagatagggtctctcactatcttcatttaagcagtgagacaaagttgcttgagaaagtgcaacatgagttgttgtctgtgtatgccactcaacttcttgagaaggagcactctgggtgccatgcgttactaagagatgataaggttgaagatttatcaaggatgtataggctcttttctaagattcctcgaggcttagaccctgtggctaatatatttaagcagcatgttactgctgaaggtacagctttggtcaaacaggctgaagatgctgctagcaacaaaaaggcagagaaaagagatgtggttggtttgcaggaacagatttttgttcggaaagtgattgagcttcatgataagtatatggcatatgtgaataactgtttccaaaaccacacactttttcacaaggcgcttaaagaagctttcgaacttttctgcaacaagggtgttgctggtagctcaagtgctgaacttcttgccacattctgcgacaatattctcaagaaaggcgggagtgagaaattgagtgatgaagccattgaagagacgctggagaaggttgtaaagctgctagcatatattagtgacaaggacttgtttgcagaattctataggaaaaagctagcccggcggttgttatttgataagagtgccaatgatgaacacgagagaagtatccttacaaagttgaagcagcagtgtgggggccagttcacatcaaagatggagggaatggtgacagatttgacattggcaagggaaaatcaagccagctttgaggagtatttgagcaacaatccagcagcaaatccaggaattgacttgacggtgactgtcttgactactggcttctggcctagctacaagtcttttgatctcaacctcccagcagaaatggttaggtgcgttgaagtattcaaggagttttatcaaacaaaaacgaagcacaggaaacttacgtggatatactctttgggaacttgcaatataaatggaaaatttgagccaaagactattgagctcgttgtcactacttatcaggcttctgctctgctgctctttaatgcatcggatagattgagttatcaggaaatcatgacgcaactaaacctatcagatgatgatgttgttcggcttcttcattccctttcatgtgcgaagtacaagattctcaacaaggagccaagcaccaaaacaatttctccgactgatgtctttgagttcaattttaagttcactgacaaaatgaggaggatcaagatacctctccctcctgttgatgagaagaaaaaggtaattgaagatgttgacaaagataggcggtacgctatagatgcttcaattgtgcgtattatgaagagtcgtaaagtattgggctaccagcaactggtcatggagtgtgttgagcagttgggacgtatgttcaagcctgatgtcaaagctatcaagaagagaattgaagatttgataactagagattacctagagagggacaaagataatccgaacttgttcaagtacttggcatga

SEQ ID NO: 8 - DNA, 2217 bp, Brassica oleracea
  source 1..2217: /organism="Brassica oleracea" /mol_type="unassigned DNA"
atggagcgcaagacgattgacttggaccaaggatgggactatatgcagactggtatcactaagctgaaacggattcttgaggggctgcctgagccgcagtttgactctgagcaatacatgatgctctatacgactatctacaacatgtgcactcagaaacctcctcatgattactcacagcagctttatgacaagtatcgtgaagcatttgaggagtatattcactcaactgttttgcctgctctaagggagaagcatgatgagtacatgctgagggagctggttaagagatggtctaaccataaagttatggttcgatggctatcccgcttcttctactatcttgaccgttacttcattgctcggaggtcacttccacccctgaatgaagttggcctgacttgcttccgtgacctggtttataacgagttgcattccaaggtcaaagatgctgtaatagcacttgttgataaagaacgggagggtgagcagattgacagggctctattgaaaaacgtattagacatttatgtagagattggaatgggacagatggaaagatacgaggaggattttgaaagcttcatgcttttagattcagcatcttactattctcgcaaggcgtcaagctggatccaagaagattcttgccctgattacatgctgaagtctgaagaatgtcttaagaaggagagggagagagtggctcactaccttcactcaagcagcgagccaaagctggttgagaaagtacaacatgagctgttggtagtgtatgcaaatcagcttctagaaaaagagcattcagggtgccgtgcattgctgagagatgacaaggttgatgacctctccaggatgtacaggctttatcataaaattgtgaaaggtttggaacctgttgcaaacatatttaagcagcatgtcacagcagagggtaacgcacttgtccaacaggccgaagacacggccactaatcatgctgcaaatactgctagcgtgcaggaacaggttcttatcagaaaagtgattgaactacatgataaatacatggtctatgttgttgagtgtttccagaaccacaccctcttccacaaggcattgaaagaggcatttgagatattctgtaacaaaacagtcgctggaagttctagtgctgaattgcttgcaacattttgcgacaatattctcaagaaggggggaagtgaaaagctgagcgatgaagctattgaagatacccttgagaaggtggtcaaattgcttgcttatataagtgacaaggatcttttcgccgagttctacaggaagaagctggcccgtaggctcttatttgatcgcagtgctaatgatgatcatgagagaagtatcctgacaaagctcaagcaacaatgtggtgggcagtttacttcgaagatggagggcatggtgactgatttgacattggcaagggaaaaccaaaacagcttcgaggagtatcttggcaataaccccgctgcaaacccagggattgatttgaccgtaactgttcttaccactggtttttggccaagttacaaatcatttgacataaatctacccgctgaaatggtcaagtgtgttgaagttttcaaagggttttatgaaacaaagacaaaacataggaaacttacctggatctactcactaggaacttgccacctcaatgggaagtttgatgtcaagcccattgagttagttgtgtctacataccaggctgctgtgcttctgctgttcaacacaacagacaaattgagctacactgatatcctaactcagctgaacctgagccacgaagatctagtgaggttgcttcattccttgtcatgtgctagatacaagattcttctcaaggagccaagcacaaagactgtttcccagtctgattcttttgaattcaactccaaattcaccgacagaatgcggagaataaagatccctctcccacctgttgatgagaggaagaaagttgtggaagacgtggacaaagacagacgctatgcgattgatgctgccattgtgaggatcatgaagagcaggaaagtattgggacatcaacaacttgtttctgagtgcgttgagcaacttagccgaatgttcaagcctgatatcaaggcaatcaagaagcgcatggaggatttgataacgagagattatctggagagggacaaggagaacgctaacatgtttaggtacttggcttag

SEQ ID NO: 9 - DNA, 2232 bp, Daucus carota
  source 1..2232: /organism="Daucus carota" /mol_type="unassigned DNA"
atgatgattgagcggaaaactatagacctggagcagggatgggactttatgcaaaagggaatcacaaagctaaagaatattttagaaggctttccggagccgcaattcagctcggaggattatatgatgctttatacaactatctataacatgtgtacacagaaacctccacatgattactctcagcagctgtatgaaaagtatcgtgaagctattgaggagtacattacttctacagtattgccttcattgagagagaagcatgatgaattcatgcttagagaacttgtgaagagatggtctaatcataaggtcatggtcaggtggctttctcgattctttcactatcttgatcgctattttattgctcggaggtcacttccaccacttcatgaagttggactcacttgctttcgggacctggtttaccaggagataaatgggaaagtaagggatgctgtaatatcattgattaatcaagagcgcgagggagagcaaattgaccgagctttgttgaagaatgttctagatatatttgttgaagttggaatgagtcaaatggattattatgagaatgactttgaagcagacatgctcaaagatacagcagcatactattctcgaaaggcttccaactggatcttagaagattcttgtccagattatatgctcaaagcggaagagtgtttgagacgggaaaaggacagggtctctaactaccttcattctagtagtgaacccaagttgcttgagaaagttcaacatgagttactatcacactatgcaactcagctgcttgagaaagaacactctgggtgtcatgcattgcttagggatgacaaggtggcagatttatcaaggatgtataggctcttctctaaaatacctcgaggcctagatcccgtgtctaatattttcaagcagcatgttactgctgaaggtacagctttggtcaaacaagcagaagatgcagctagcaacaagaaggcagagaagagagatgtagtaggtttacaagaacaggtttttgtgaggaaaataattgaattgcatgacaaataccttacatacgtaaatgactgttttacaaaccacactctcttccataaggcgcttaaggaggcttttgaaatcttctgcaataagggtgtctctggaagctctagtgcagaattacttgccacattctgtgataatattctcaagaaaggtggaagcgagaagttaagtgatgaagccattgaggaaacacttgagaaggttgtaaggttgcttgcttatataagtgacaaagacttatttgctgaattttataggaaaaagcttgcacggcgtctcttattcgacaagagtgccaatgatgagcatgagagaagtatattgactaagctgaagcaacaatgtgggggtcaatttacatcaaagatggaaggaatggtcactgacttgacgttggcaaaggaaaatcagtccaacttcgaggagtacctcaataataattcaaacgtaaatcctggaattgacttgacagttactgttctaaccactgggttttggccaagttacaaatctttcgatctcaacctcccagcagagatggtcaaatgtgttgaagtttttagagaattctaccaaacaaaaacaaagcacagaaaactgacatggatatactctttgggtacttgtaacatcattggaaaatttgatccaaaaaccatggagcttattgtgacaacataccaggcctctgctctgctgctatttaactcttctgatagacttagttataatgaaataatgactcagttgaacttgtcggatgatgatgttgtcagactacttcattctctttcgtgtgcaaagtacaagattctatctaaagagccgaacaccaaaactatatctccaactgattgctttcagttcaattccaaatttactgataaaatgaggaggattaagattccacttcccccagtggatgagaagaaaaaggtaattgaagatgttgataaagacaggcgatatgctatagatgcttcaattgtccgtatcatgaagagccgcaaagttttgggttatcagcagctagtaatggagtgcgttgaacaattgggtcgcatgtttaagcctgatgtcaaagcaatcaagaagagaatcgaagatttaataactcgggattatctggaaagagacaaggacaatgccaacttgttcaggtatctggcatga

SEQ ID NO: 10 - DNA, 2229 bp, Apium graveolens
  source 1..2229: /organism="Apium graveolens" /mol_type="unassigned DNA"
atgaacgagcggaagactatcgatttggataatggatgggaatttatgcagaaagggatcactaagttgaagaagattctcgaaggtcaacctgagcctcagtttagctccgaggactatatgatgctttacacaactatctataatatgtgtacgcagaagcctccacatgattattctcaacagctgtatgacaagtaccgtgaggcctttgaggagtacataacttcaactgtcctgccttctttacgagagaagcatgatgagtttatgttgagagagctcgtgaatagatggacaaaccataaagtcatggtcaggtggctttctcgattctttcactatcttgatcggtacttcattgcgaggaggtcacttcctgcacttcatgaagttggactcacgtgcttccgggatctggtctatcaggagctgaaagttaaagtgagggatgctgtaatatctctgatcgatcaagagcgtgagggggaacagattgaccgagctttattaaagaacgtgttagatatatttgttgaaatcggaatgagtcaaatggatcaatatgagaatgactttgaagaagccatgctcactgatactgctgcttactattctcgaaaagcttcaaactggatccttgaagattcttgtcctgattatatgttaaaggcagaagaatgtttgcgacgagagaaggacagggtttcccactacctacattttagtagcgagccaaagttgcttgagaaagtgcaacatgagctgctatctgtgtatgcaacccaattactcgagaaggaacattctggttgtcatgcattgcttagggatgacaaggtggatgatttgtctaggatgtacagactcttctcgaaaatacctaaaggcctggatccagtttcttatatttttaagcagcatgttacaaatgaagggatggcattggttaaacaagcagaagatgcagcaagcaacaagaaggcagaaaagagagacgtggttagtttacaggagcaggtttttgttagaaaaattattgaattacatgacaaatacctcgcctatgtgaatgactgctttacaaaccatactcttttccataaggctctcaaggaggcttttgaaatcttttgcaacaagggtgttgctggaagctctaatgctgaactacttgctactttctgtgataacatcctcaaaaagggtgggagtgagaaattaagtgatgaggctattgaagaaacacttgagaaggtagtaaaattgttagcttacattagcgataaagacttgttcgctgaattttacagaaaaaagcttgcacggagacttctctttgataagagtgcaaatgacgagcatgaacgaagtattttgactaaactaaagcaacagtgcggtggtcagttcacatcgaaaatggaggggatggtcacagatttgactttggctaaagaaaatcaatccagctttgaggagtatctgggaaataatgccaatgtgaatcctggcattgacttgacggttactgttctgaccactggcttctggcctagttataaatcctttgatctcaaccttcctgctgagatggtcaagtgcgttgaagtatttagagaattttatcaaacaaaaacgaagcatagaaagctcacatggatatattctctgggtacttgtaatatcaatggaaaatttgaacccaaaaccattgagctgattgtgacaacctaccaggcctctgctctcctgttatttaatacttctgataggttgagttatcaagaaatcatgactcagttaaatttgtcggatgatgatgttgttcgcctgcttcattccctttcatgtgccaagtataaaattcttactaaagagccgaacaacaaaacaatttcccctacggattactttgagttcaactccaagttcactgacaaaatgaggagaattaagattccactacctccagttgatgagaagaaaaaggtaattgaagatgttgacaaggaccggcgatatgccattgatgcatctattgtccgcattatgaagagccgtaaagttttgggctaccaacaattggttatggaatgtgttgagcaattgggacgcatgtttaagcctgatgtcaaagcaattaagaagagaatcgaagatttaataacgcgtgattatctggaaagagacaaggataatgccaaccttttcagatatttggcatga

SEQ ID NO: 11 - DNA, 2229 bp, Cichorium intybus
  source 1..2229: /organism="Cichorium intybus" /mol_type="unassigned DNA"
atgaatgaaagaaaaacaatagacttagaacaaggatgggacttcatgcagaaaggcataacaaagttgaagaacattctagaaggtcttcccgagccacaattcagctcggaagattacatgatgctctacacaaccatctacaatatgtgcacacaaaaaccgccacatgattactctcaacaattgtatgacaaataccgcgagtcttttgaagagtacattacttcaacggtgttaccttctttaagagagaagcatgatgagtttatgcttagagagcttgttagaagatggtcaaatcataaagtgatggttaggtggctttctagattcttccattatcttgatcgatacttcattgcccgaagatctcttccaccattaaatgaagttggacttgcgtgttttcgtgatctggtataccaagaggtgaatgggaaagtgagagatgctgtaatatctttgattgatcaagagcgtgaaggcgagcaaattgaccgagcattactcaagaatgttctagatatatttgttgaaataggaatgggacaaatggaatattatgagaatgattttgaagcatccatgcttaatgatacagcagcatattattcacgcaaagcttccaattggattctagaagattcttgtccagattatatgctcaaagctgaggagtgcttaaaaagagaaaaggacagagtttctcattatcttcattccagcagtgaaccaaagcttcttgagaaagttcaaacagagttattatctgtttatgcaactcaattgcttgaaaaggagcactccggttgtcatgcattacttagggatgacaaggttgatgatttatcaagaatgtacagactcttttcaaagatacaaaaagggctggatcctgtttctagtatgtttaagcagcatgtcactgctgaaggcacaacattggttaaacaggcagaagatgcagcaagtactaagaaggctgaaaagagagacgtggttggcttacaagaacaggtttttgttagaaaagttatcgagcttcatgacaagtaccttgcatatgtaaatgactgttttatgaatcataccctgtttcacaaggctcttaaagaggcatttgaaatattctgcaacaagggcgttgctggaagttcaagtgcagaattacttgctacattttgtgataatattcttaaaaaaggtggaagtgaaaaattgagtgatgaagccattgaggacacacttgagaaggtggtaaagttgcttgcttacatcagcgataaagatctatttgcagagttttataggaaaaaactggctagacggcttttatttgacaaaagtgcaaatgatgagcacgaaagaagtattttgacaaaattgaaacaacaatgtggcggtcaatttacatcaaaaatggaaggaatggttacagatttgacattggcaaaagaaaatcaatcacattttgaggagtatttgaataataatcccaatgttagccctggcattgacttgaccgtgactgtgttgaccactggtttttggcctagttacaaatcttttgacctaaatctccctgcagaaatggtcaaatgcgttgaagttttcagagaattttatcaaacaaaaacaaaacacagaaaactcacatggatatattcattgggcacctgcaatataaacggaaaattcgaaccaaaaaccatggagctaatcgttacaacttaccaggcatctgctttattactgttcaactcatcagatcgattgagttatcaagaaatcatgactcaattaaacttatcagatgatgatgttgttagactactccattcattatcatgtgcaaaatataaaattttattaaaagaaccaaatacaaaaacaatctctccaactgatttctttgaattcaactcaaagtttacagataaaatgagaaggatcaagattcctctacctcctgttgatgaaaagaaaaaagtaattgaagatgttgacaaagaccgacgttatgcaattgatgcttcaattgtacggataatgaaaagcagaaaagttcttggataccaacaattggtcatggaatgtgttgaacaattaggccgtatgtttaagcctgatgtaaaagcaatcaagaaacgtattgaagatctcataactcgtgattatcttgaaagagacaaagaaaatccaaatttgtttcggtacttggcatga

SEQ ID NO: 12 - DNA, 2229 bp, Cichorium endivia
  source 1..2229: /organism="Cichorium endivia" /mol_type="unassigned DNA"
atgaatgaaagaaaaacaatagacttagaacaaggatgggacttcatgcaaaaaggcataacaaagttgaagaacattctagaaggtcttcccgagccacaattcagctcagaggattacatgatgctctacacaaccatctacaatatgtgcacacaaaaaccgccacatgattactctcaacaattatatgacaaataccgcgagtcttttgaagagtacataacttcaacggtgttaccttctttaagagagaagcatgatgagtttatgcttagagagcttgttagaaggtggtcaaatcataaagtgatggttaggtggctttctagattcttccattatcttgatcgatactttattgcaagaagatctcttccaccattaaatgaagttggacttgcgtgttttcgtgatctggtataccaagaggtgaatggaaaagtgagagatgctgtaatatctttgattgatcaagagcgtgaaggcgagcaaattgaccgagcattactgaagaatgttctagatatatttgttgaaataggaatgggacaaatggaatattatgagaatgattttgaagcatctatgcttaatgatacagcagcatattattcacgcaaagcttccaactggattctagaagattcttgtccagattatatgctcaaagctgaggagtgcttaaaaagagaaaaggacagagtttctcattatcttcattcaagtagtgaaccaaagcttcttgagaaagttcaaacagagttattatctgtttatgcaactcaattgctcgaaaaggaacactcaggttgtcatgcattacttagagatgacaaggttgatgatttatcaagaatgtacagactcttttcaaagatacaaaaaggactggatcctgtttccagtatgtttaagcagcatgtcactgctgaaggcacaacattagtaaaacaagcagaagatgcagcaagtactaagaaggctgaaaagagagacgtggttggcttacaggaacaggtttttgttagaaaagtaatcgagcttcatgacaagtacctcgcatatgtaaacgactgttttatgaatcacacattgttccacaaggctcttaaagaggcatttgaaatattctgcaacaagggcgttgctggaagttcaagtgcagaattacttgccacattttgtgataatattcttaaaaaaggtggaagtgaaaaattgagtgatgaagccattgaagacacacttgagaaggtagtaaagttgcttgcttacatcagcgataaagatctatttgcagagttttataggaaaaaactggctagaaggcttttatttgacaaaagtgcaaatgatgagcatgaaagaagtattttaacaaagttgaagcaacaatgtggtggtcagtttacatcaaagatggaaggaatggttacagatttaacactggcaaaagaaaatcaatcacattttgaggagtatttgaataataatcccaatgttagccctggcattgacttgaccgtgactgtgttgaccacgggattttggcctagttacaaatcttttgacctaaatcttcctgcagaaatggtcaaatgcgttgaagttttcagagaattttatcaaacaaaaacaaaacacagaaaactcacatggatttattcattgggcacctgcaatattaacggaaaattcgaaccaaaaaccatggagctaatcgttacaacttaccaggcatctgctttattgttattcaactcatcagatcgattaagttatcaagaaatcatgactcaattaaatttatcagatgatgatgttgttagactactacattcattatcatgtgcaaaatataaaattttattaaaagaaccaaataccaaaacaatatctccaaccgatttctttgaattcaactcaaagtttacagataaaatgagaaggatcaagattcctctacctcctgttgatgaaaagaaaaaagtaattgaagatgttgacaaagatagaaggtatgcaattgatgcttcaattgtacgaataatgaaaagcagaaaagttcttggataccaacaattggttatggagtgtgttgaacaattaggccgtatgtttaagcctgatgtaaaagcaatcaagaagcgtattgaagatttgataacgcgtgattatcttgaaagagacaaagaaaatccaaatttgtttcggtacttggcatga

SEQ ID NO: 13 - DNA, 2235 bp, Allium ampeloprasum
  source 1..2235: /organism="Allium ampeloprasum" /mol_type="unassigned DNA"
atgtcgttgcacgaaaggaaaaccattgatttggagcagggatgggcttttatgcagaaagggatcaccaaactgaagaatattcttgatgagttgaatgaacctcagttcagctcagaggattacatgatgctctatacgactatctataatatgtgtactcagaagccgccacatgattattctcaggagttgtatgataagtaccgagagtcctttgaagagtatatcactaccactgtgcttccttcattgagagaaaagcatgatgaatacatgttaagggagctcgtgagaaggtggtcaaatcataaaataatggttagatggctttcacgctttttccattatcttgatcgctactttatagcacgaagatcattgcctgctcttaatgaagtcggtctcacttgtttccgtgatctggtgtacaacgaagtccatgggaaagttaaagatgccgtgatctcattgattgaccaagagagggaaggggagcaaattgacagagctttattaaagaatgttttgggtatttttgtagagattggtttgggaagcatggaatgttatgagaatgattttgaaacatcaatgcttaatgctacagcagcctattattcacgaaaagcttcaaattggattctagaagattcatgtccagattatatgctaaaagccgaggagtgcttaaaacatgagaaagatagagttgctcattatttgcattcaagcagtgaacagaagctgttagagaaagtgcaacatgagttacttttcgtatatgcaagtcaacttctcgagaaagaacattccggatgtcatgcattgcttcgcgatgacaaggtgggagatctttcacgcatgtatcggctgttctgtagaattacacgtggtttggaccctgtgtctcaaatatttaagcagcatgtgactgcagaaggtactgctttggtcaaacatgccgaagatgctgcaagtaacaagaaggccgagaaaaaagacattgttggtttgcaagagcaggtcttcgttaggaaagtaattgagctgcatgataaatacttggcctatgtgactgactgctttcaaaatcactctctatttcacaaggcacttaaagaggcattcgaggtattctgcaataaaggtgttgcaggtagctcaagcgctgaacttctggctgctttttgtgacaatatattgaagaagggtggaagcgagaaactaagcgatgaggccatagaggatactcttgagaaggttgtaaaactattggcatatattagcgataaagatctgtttgctgaattttacaggaagaagcttgcacgaagattactctttgacaaaagtgctaatgatgaccatgagaggagcatccttacaaagctgaaacagcaatgtggagggcagttcacctctaaaatggaaggcatggtaaccgatctgacacttgcacgagaaaatcaatcaagttttgacgattaccttagcagcaatcctaaagcaaattctggaattgacttgactgttacagtcttaacaactggcttctggcccagttacaagtcttttgatctcaatcttcctgatgagatggtaaaatgcgttgaaatttttaaagagttttacgagacaaaaaccaaacacagaaaacttacatggatttattcgttgggcacttgcaacatcaatggcaagttcgaaaccaagacaatagagttggttgttacaacctatcaggctgcagtgttgcttctattcaactctgcagataaattaagttattctgagattgtgcagcagctaaacttatctgatgatgatgtaatcagattacttcactctctttcatgcgctaaatacaaaattctcaataaagaacccgctaccaagactattaccccgaatgatcattttgagttcaattctaaattcactgatagaatgagaaggatcaagattcccctgcctcctgtggatgagaagaaaaaagtaattgaagatgttgacaaagacagaagatatgcaattgacgcatccatagttcgaataatgaaaagtagaaaagttcttggtcatcagcagcttgttttggaatgtgttgagcaattaggccgcatgtttaagcctgactttaaggccatcaagaaaaggattgaagatctgatcgctagagattatttggagagggacaaggacaatccaaacctctttaaatatttggcctaa

SEQ ID NO: 14 - DNA, 2229 bp, Lactuca sativa
  source 1..2229: /organism="Lactuca sativa" /mol_type="unassigned DNA"
atgaacgaaagaaaaacaatagacttagagcaaggatgggacttcatgcagaaaggaataacaaagttgaagaatattctagaaggtcttcccgagccacaattcagctcggaggattacatgatgctctacacaaccatctacaacatgtgtacacagaaaccaccacatgattactcccaacagttgtatgacaaatatcgtgagtcttttgaagagtatattacttcaactgtgttaccttctttaagagagaagcatgatgagttcatgctgagagagcttgttagaaggtggtcaaatcataaagtcatggtgcggtggctttctagattcttccattatcttgaccgatatttcattgcccgaagatctcttccgccactaaatgaagttggacttgcctgttttcgtgatctggtataccaagaggtgaatggtaaagtgagagatgctgtaatatctttgattgatcaagagcgtgaaggggagcagattgatcgagctttactgaagaatgttctagatatatttgttgagataggaatgggacaaatggagtattatgagaatgattttgaagcatccatgcttaatgatacagcagcatattattcacgcaaggcttccaactggattctagaagattcttgtccagattatatgctcaaagcagaggagtgcttaaaaagagaaaaggacagagtgtctcattatcttcattccagcagtgagccaaagcttcttgagaaagttcaaaatgagttattgtctgtttatgcaactcaattgcttgagaaagagcactcaggttgtcatgcattgctcagggatgacaaggttgatgatttatcaagaatgtacagactcttttcaaagataccaaaaggattggatcctgtttctagtatgtttaagcagcatgtcactgctgaaggcacaacattggttaaacaagcagaagatgcagcaagtaccaagaaggctgaaaagagagatgtggttgggttgcaggaacaggtttttgttagaaaagttattgagctccatgacaagtacctggcatatgtaaatgactgtttcatgaaccatactcttttccacaaggctcttaaagaggcatttgaaatattctgcaacaagggtgttgctggaagttcaagtgcagagttacttgccacattttgtgataatattcttaaaaaaggtggaagtgagaaactgagcgatgaagccattgaggacacccttgagaaggtagtaaagttgcttgcctacatcagtgataaagatctatttgctgaattttacaggaaaaaacttgctaggaggcttttgtttgacaagagtgcaaacgatgagcatgagagaagtattctcacaaagctgaagcaacagtgtggtggtcagttcacatcaaagatggaagggatggttacagatttgacattggcaaaggaaaaccaatcccattttgaagagtatttgaacaataatcccaatgtcagccctggaattgacttgactgtcactgtgttgactaccggcttctggcccagctacaaatcttttgacctaaatctccctgccgaaatggttaaatgcgttgaagttttcagagaattttatcaaacaaaaacaaagcacaggaagcttacatggatatattcattgggtacctgcaatataaacgggaaatttgaacccaaaacaatggagctcatagtcacaacctaccaggcatctgctttattactgttcaacttatcggatcgattgagttatcaagaaatcatgactcagttgaacttgtcagatgatgatgttgttaggctgctccattctttgtcatgtgcaaaatacaaaattcttttaaaggagcctaataccaaaacaatctctccaaccgattacttcgaattcaactccaagtttacagataaaatgaggaggatcaagattcctctacctcctgtggatgagaagaaaaaggtgattgaggatgttgacaaagacagacgttatgccattgatgcttccattgtaaggataatgaagagcagaaaggtgcttggataccagcagttggttatggagtgtgttgaacagttgggacgcatgtttaagcctgatgtaaaagcaatcaagaagcggattgaagatctgataactcgtgattatcttgaaagagacaaagagaaccccaacttgttccgatacttggcatga

SEQ ID NO: 15 - DNA, 2217 bp, Raphanus sativus
  source 1..2217: /organism="Raphanus sativus" /mol_type="unassigned DNA"
atggagcggaagacgattgatctggaacaaggatgggactatatgcagactgggatcactaagctgaaacggattcttgaaggattgcctgagccgcaattcgactctgagcagtacatgatgctttatacgactatctacaacatgtgcacccagaaacctcctcatgattactctcagcagctttatgacaagtatcgcgaagcttttgaggagtacattgactctactgttttgcctgctttgaaggagaagcatgatgaatacatgctacgggagctggttaagagatggtctaaccataaagttatggttagatggctatcccgattcttctactatcttgaccgttacttcattgctcggagatcgctgccaccgcttaatgaagttgggctcacatgcttccgtgaccgggtgtataaggagttgcattccaaggtcaaagatgctgtaatagcacttgttgataaagaacgggaaggcgagcagattgacagggctcttctgaaaaacgtattagatatctatgtagagattggaatgggacagatggaaagatacgaagtggattttgaaagcttcatgcttttggattcagcatcttactattctcgcaaagcatcaaactggatccaggaagattcttgccctgattacatgctgaagtctgaagaatgccttaagaaggagagggagagggttgctcactaccttcattcaagcagcgagccaaagctggttgagaaagtacaacatgagctgttggttgtctatgcaaatcagcttcttgaaaaggagcactcagggtgccgtgcattgctgagagacgacaaggttgacgatctctccaggatgtacaggctctatcataaaattgctaaaggtttagaacctgttgcaaacatatttaagcagcatgtcacagccgagggtaacgcacttgtccaacaggccgaagacacagccactaatcaggctgcaaatactgctagcgtgcaggaacaggttctcatcagaaaagtgattgagctacatgataagtacatggtctatgtcgtggagtgcttccagaaccacaccctcttccacaaggctctgaaagaggcatttgagatattctgtaacaaaacagtcgctggaagttcaagtgcagaactgcttgcaacattctgcgacaacatcctcaagaaggggggtagtgagaagctgagtgacgaagctattgaagatacgcttgagaaggttgtcaaattgcttgcttatataagcgacaaggatcttttcgccgagttctacaggaagaagctggcacgtaggctcttatttgatcgcagtgcgaatgatgatcatgagagaagcatccttacaaagctcaagcaacaatgtggtgggcagttcacttctaagatggagggcatggtaacggacttgacattggcaagagagaaccaaaccagtttcgaggagtatctaggcaataaccccgctgcaaacccagggattgatttgaccgtcactgttcttaccactggtttctggccaagttacaaatcattcgacataaatctaccaagtgaaatggtcaagtgtgttgaagttttcaaagggttttatgagacgaaaactaaacataggaaacttacatggatctactcactaggaacttgtcacctcaacggaaagtttgatcacaagcccattgagttagttgtgtctacttaccaggctgctgtgcttctgctgttcaacacaacagacaaattgagctacaacgatatcctaactcaactgaacctaagccacgaagatttagtgaggttgcttcattccctgtcatgtgctaggtacaagatccttctcaaggagccaagcacgaagactgttacacagactgattcatttgaattcaatgccaaattcacggacagaatgcgcagaatcaagatccctctccctcctgttgatgaaaggaagaaggttgtggaagatgtggacaaagacagacgctatgcgattgatgctgccattgttaggatcatgaagagcaggaaagtgttgggacatcaacaactcgtctctgagtgcgttgagcaacttagccgaatgttcaagcctgatatcaaagcgatcaagaagcgtatggaggatctaattacgagggattatttggagagggacaaggagaaccctaacatgtttaggtacttggcttag

SEQ ID NO: 16 - DNA, 2223 bp, Spinacia oleracea
  source 1..2223: /organism="Spinacia oleracea" /mol_type="unassigned DNA"
atgaacgatcgtaaagttatcgaactagagcaaggatgggagttcatggggaaggggattacgaagttgaaaaggattttggaaggattaccagagccgccttttaattcggaagactacatgatgctgtacacgacaatatacaacatgtgtacacagaaaccccctcatgattactctcaacaactctatgacaattacaaagaggcatttgtggattacatacattcaacggttttaccttctttgggggacaaacatgatgagtttatgctgagagagcttgtgaagagatggtcaaatcataaagtaatggtgaggtggttgtctcgcttcttccattatctggatcggtacttcatcgctcggagatcgcttccttctttgaatgatgttggattgacgtgcttccgtgatctggtttatcaagaaatatctggcaaagccaaggatgctgttattgctctgattgatgaagaaagagagggtgggcaaattgacagagccttattgaagaatgtacttgatatatacgttgaaattggaatgacacaaatggattactacgaaaaggactttgaagctcatatgctggatgatactgctgcttattactcacgcaaggcctcaagctggattctggaggactcatgtccggaatacatgttgaagtcggaggagtgtttgaagaaagagaaagatagagtggctcattatctacattccagcagtgagccaaagcttctggagaaagtacaaaatgagttgctactggtttacgaaaatcagttgcttgagaaggagaattctggatgtcgtgcattgttgaaagatgacaaggtggaagatctttccaggatgtacaggctttatagcaaggttaccaaagggttggaacccattggcagtatcttcaaacagcatataaccgatgaaggaacagccctggtgcagcaggccgaagacgctgcaattagcaaggctgaaaatgctggcggtggttcacatgagcaggtcttcgtcaggaaagtgattgagttgcatgacaaatttatgacctatgttacagattgcttcaacagccataccatctttcacaaggctctcaaggaagcttttgaggtattcttaaacaagggtgttgctggtagttcaagtgctgaacttctagcttcattttgtgataatattctcaagaaaggtggtagtgaaaaattaagtgatgaggctattgaggattcactggagaaggtggtgaagcttctcgcatatgtcagtgataaagacctgtttgctgaattttacagaaagaagctctctcgccggctactctttgacaaaagtgctaatgatgatcatgagaggagtattttaacaaaattgaagcagcagtgtgggggacagttcacatcaaagatggaggggatggtgacagacttgacattggcgagggagaatcaaactaattttgaggaatatcttggacaaaatacagatgccagtcctggtcttgatttgactgtgacagttttgaccactgggttctggccaagttacaaatcttctgatcttaaccttcctgctgagatggtgaggtgtgttgaagtttttaagcaattttatcaaacaaagacaaaacacaggaagctcacctgggtatattcgttgggaagttgtaacattaatggcaagtttggtccgaaaacaattgaattggttgttggaacttatcaggctgctgcgctgatgctctttaacacatcagatcgactgagttattcagaaataacgacccaactaaatctagctgacgaagacttggttagagtgcttcaatctctatcttgcgcaaagtataagattcttctaaaagagccaagcacaagaaacgtgatctcaactgattgtttttcattcaactctaattttactgacagaatgaggaggattaggattcctcttcctccaatggatgagaggaaaaaggttgttgaagatgttgacaaagatagaagatatgctattgatgcctcaattgtacgcataatgaaaagtaggaaggctttgggatatcaacaattaatcacggagtgtgtggagcagctaagccgcatgttcaagcctgatttcaaagcaattaagaagaggatcgaggacttgataaccagagattatattgaaagagacaaggaaaaccctcagctattccggtacttggcttga

SEQ ID NO: 17 - DNA, 2220 bp, Beta vulgaris
  source 1..2220: /organism="Beta vulgaris" /mol_type="unassigned DNA"
atgaatgatcgtaaagttattgaactagagcaaggatgggagttcatggggaaggggattacaaagttgaagaggattctggaaggattgccagagccaccatttaattctgaagactacatgatgttgtacacgacgatatacaatatgtgtactcagaaacccccacatgattactctcaacagctctatgacaattacaaacaggcttttgtggattacatcaactcgacggttttaccttctttgcgggagaagcatgatgagtttatgttaagagaacttgtgaaaagatgggcaaatcataaagtaatggtcaggtggttgtctcgtttcttccattatctggaccggtatttcattgctcggaggtcgcttccttctttgaatgaagttggactgacttgtttccgtgatctggtttatcaagaaatatctggcaaagccaaggatgctgttatagccctgattgatatagaaagagaaggtgggcagattgacagatcattattgaaaaatgtacttgatatatatgttgaaattggaatgggacaaatggatcactatgaaaaagactttgaagctcatatgctggatgatactgctgcttactactcgcgcaaagcgtctagctggattcttgaggactcttgtccggaatacatgttaaagtctgaggagtgtttgaagaaggagaaagagagagtggctaattatttacattccagcagtgagccaaagcttctggagaaagtgcaaaacgagttgctattggtttatgaaagccaattgcttgagaaggagaattcgggatgtcgtgcattactgaaagatgacaaggtggatgatctttccaggatgtacaggctttacagtaaggttaccaaaggattggaacccattggcagtatcttcaaacagcatataactgatgaaggaacagccttagtgcagcaggccgaagatgctgctatcagcaaggctgaaaatactggtggttcacatgagcaggtcttcgtcaggaaagtaatagagttgcatgacaaattcatgacttatgtcaccgattgcttcaacagccataccatatttcacaaggctcttaaggaggcttttgaggtatttttgaacaagggtgttgctggtagctcaagtgctgagttgctagctacattctgtgataacattctcaagaaaggtgggagcgaaaaactaagcgatgaggctattgaggattcacttgagaaggtggtgaagcttctggcctatgtcagtgataaagacctgtttgctgaattttacagaaagaagctctctcgccggctactctttgacaagagtgctaatgatgatcatgaaagaagtattttaaccaaattgaagcagcagtgtggcggacaattcacatcaaagatggaggggatggtgacagacttgaccttggcgagggagaatcaaactaattttgaggaatatcttagtcagaatccagatgccagtcctggtcttgatttgactgtgactgttctgacaactgggttctggccaagttacaaatcttccgatcttaaccttcccgctgagatggtgaggtgtgttgaagtttttaagcagttctattcaactaaaacaaagcacaggaagctgacctgggtttactcattgggaagctgtaatattaatggcaagtttggtccaaaaactattgaattggttgtcggaacttatcaggctgctgctttgatgctctttaacacatcagaccgactgagttattcagagatagcaactcaactaaatttagctgatgaagatctggttagagtgcttcaatctttatcctgcgcaaagtataagattcttttaaaggagccaaacacgaaaaccgtgtccccgactgattgtttttcatttaactctagtttcactgacaggatgaggaggataagaattcctcttcctccgatggatgagaggaaaaaggttgttgaggatgttgacaaagatagaagatatgctattgatgcctcaattgtacgcataatgaaaagtaggaaggttttggggtaccagcaattaatcacagagtgtgtggagcagctaagccgcatgttcaagcctgatttcaaggcaattaagaagaggatcgaggacttaataacccgagattatattgaaagagacaaggagaacccgcagctattccgatacttggcttga

SEQ ID NO: 18 - protein, 744 aa, Cucumis sativus
MTMGERKTIDLEQGWEFMQKGITKLKNILEGLPEPQFSSEDYMMLYTTIYNMCTQKPPHDYSQQLYDKYRESFEEYITSMVLPSLREKHDEFMLRELVKRWTNHKVMVRWLSRFFHYLDRYFIARRSLPPLNEVGLTCFRELVYKELNSKVRDAVISLIDQEREGEQIDRALLKNVLDIFVEIGMGQMDYYENDFEAAMLKDTAAYYSRKASNWILEDSCPDYMLKAEECLKREKDRVSHYLHSSSEPKLLEKVQHELLSVYATQLLEKEHSGCHALLRDDKVEDLSRMFRLFSKIPKGLDPVSNIFKQHVTAEGTALVKQAEDAASNKKAEKKDIVGLQEQVFVRKVIELHDKYLAYVNDCFQNHTLFHKALKEAFEVFCNKGVAGSSSAELLATFCDNILKKGGSEKLSDEAIEETLEKVVKLLAYICDKDLFAEFYRKKLARRLLFDKSANDDHERSILTKLKQQCGGQFTSKMEGMVTDLTLARENQTSFEEYLSNNPQASPGIDLTVTVLTTGFWPSYKSFDLNLPAEMVKCVEVFREFYQTKTKHRKLTWIYSLGTCNISGKFEPKTMELIVTTYQASALLLFNSSDRLSYSEIMTQLNLSDDDVVRLLHSLSCAKYKILNKEPNTKTISPNDHFEFNAKFSDKMRRIKIPLPPVDEKKKVIEDVDKDRRYAIDASIVRIMKSRKVLGHQQLVMECVEQLGRMFKPDFKAIKKRIEDLITRDYLERDKDNPHLFRYLA

SEQ ID NO: 19 - protein, 744 aa, Cucumis melo; identical to SEQ ID NO: 18

SEQ ID NO: 20 - protein, 744 aa, Cucurbita pepo
MTMGERKTIDLEQGWEFMQKGITKLKNILEGLPEPQFSSEDYMMLYTTIYNMCTQKPPHDYSQQLYDKYRESFEEYISSMVLPSLREKHDEFMLRELVKRWTNHKVMVRWLSRFFHYLDRYFIARRSLPPLNEVGLTCFRELVYKELNSKVRDAVISLIDQEREGEQIDRALLKNVLDIFVEIGMGQMDYYENDFEAAMLKDTAAYYSRKASNWILEDSCPDYMLKAEECLRREKDRVSHYLHSSSEPKLLEKVQHELLSVYATQLLEKEHSGCHALLRDDKVEDLSRMFRLFSKIPKGLDPVSNIFKQHVTAEGTALVKQAEDAASNKKAEKKDIVGLQEQVFVRKVIELHDKYLAYVNDCFQNHTLFHKALKEAFEVFCNKGVAGSSSAELLATFCDNILKKGGSEKLSDEAIEETLEKVVKLLAYICDKDLFAEFYRKKLARRLLFDKSANDDHERSILTKLKQQCGGQFTSKMEGMVTDLTLARENQTSFEEYLSNNPQASPGIDLTVTVLTTGFWPSYKSFDLNLPAEMVKCVEVFREFYQTKTKHRKLTWIYSLGTCNISGKFEPKTMELIVTTYQASALLLFNSSDKLSYSEIMTQLNLSDDDVVRLLHSLSCAKYKILNKEPNTKTISPNDHFEFNAKFSDKMRRIKIPLPPVDEKKKVIEDVDKDRRYAIDASIVRIMKSRKVLGHQQLVMECVEQLGRMFKPDFKAIKKRIEDLITRDYLERDKDNPHLFRYLA

SEQ ID NO: 21 - protein, 744 aa, citrillus lanatus; identical to SEQ ID NO: 18

SEQ ID NO: 22 - protein, 742 aa, Solanum melongena
MNQRSTIDLEHGWDFMQKGITKLKNILEGLPEPQFSSEDYMMLYTTIYNMCTQKPPHDYSQQLYDKYREAFEEYITTTVLPSLREKHDEFMLRELVKRWSNHKVMVRWLSRFFHYLDRYFIARRSLPGLNEVGLTCFRDLVYQELNGKVRDAVISLIDQEREGEQIDRALLKNVLDIFVEIGMGSMDYYENDFEAAMLKDTAAYYSRKASNWILEDSCPDYMLKAEECLKREKDRVSHYLHSSSETKLLEKVQHELLSVYANQLLEKEHSGCHALLRDDKVDDLSRMYRLFSKIPRGLEPVANIFKQHVTAEGTALVKQAEDAASNKKAEKRDVVGLQEQVFVRKVIELHDKYLAYVNNCFQNHTLFHKALKEAFELFCNKGVAGSSNAELLATFCDNILKKGGSEKLSDEAIEETLEKVVKLLAYISDKDLFAEFYRKKLARRLLFDKSANDEHERSILTKLKQQCGGQFTSKMEGMVTDLTLARENQASFEEYLSNNPTANPGIDLTVTVLTTGFWPSYKSFDLNLPAEMVRCVEVFKEFYQTKTKHRKLTWIYSLGTCNINGKFEAKTIELVVTTYQASALLLFNASDRLSYQEIMTQLNLSDDDVVRLLHSLSCAKYKILNKEPSTKTISPTDVFEFNSKFTDKMRRIKIPLPPVDEKKKVIEDVDKDRRYAIDASIVRIMKSRKVLGYQQLVMECVEQLGRMFKPDVKAIKKRIEDLITRDYLERDKDNPNLFKYLA

SEQ ID NO: 23 - protein, 742 aa, Solanum lycopersicum
MNQRSTIDLEHGWDFMQRGITKLKNILEGLPEPQFSSEDYMMLYTTIYNMCTQKPPHDYSQQLYDKYREAFEEYITTTVLPSLREKHDEFMLRELVKRWSNHKVMVRWLSRFFHYLDRYFIARRSLPGLNEVGLTCFRDQVYQELNGKVRDAVISLIDQEREGEQIDRALLKNVLDIFVEIGMGLMDYYENDFEAAMLKDTAAYYSRKASNWILEDSCPDYMLKAEECLKREKDRVSHYLHSSSETKLLEKVQHELLSVYATQLLEKEHSGCHALLRDDKVEDLSRMYRLFSKISRGLDPVANIFKQHVTAEGTALVKQAEDAASNKKAEKRDVVGLQEQVFVRKVIELHDKYLAYVNNCFQNHTLFHKALKEAFELFCNKGVAGSSSAELLATFCDNILKKGGSEKLSDEAIEETLEKVVKLLAYISDKDLFAEFYRKKLARRLLFDKSANDEHERSILTKLKQQCGGQFTSKMEGMVTDLTLARENQASFEEYLSNNPIANPGIDLTVTVLTTGFWPSYKSFDLNLPAEMVRCVEVFKEFYQTKTKHRKLTWIYSLGTCNINGKFEPKTIELVVTTYQASALLLFNASDRLSYQEIMTQLNLSDDDVVRLLHSLSCAKYKILNKEPSTKTISPTDVFEFNSKFTDKMRRIKIPLPPVDEKKKVIEDVDKDRRYAIDASIVRIMKSRKVLGYQQLVMECVEQLGRMFKPDVKAIKKRIEDLITRDYLERDKDNPNLFKYLA

SEQ ID NO: 24 - protein, 742 aa, Capsicum annuum
MNQRSTINLEHGWDFMQRGITKLKNILEGLPEPQFSSEDYMMLYTTIYNMCTQKPPHDYSQQLYDKYREAFEEYITTTVLPSLREKHDEFMLRELVKRWSNHKVMVRWLSRFFHYLDRYFIARRSLPGLNEVGLTCFRDLVYQELNGKVRDAVISLIDQEREGEQIDRALLKNVLDIFVEIGMGSMDYYENDFEAAMLKDTAAYYSRKASNWILEDSCPDYMLKAEECLKREKDRVSHYLHLSSETKLLEKVQHELLSVYATQLLEKEHSGCHALLRDDKVEDLSRMYRLFSKIPRGLDPVANIFKQHVTAEGTALVKQAEDAASNKKAEKRDVVGLQEQIFVRKVIELHDKYMAYVNNCFQNHTLFHKALKEAFELFCNKGVAGSSSAELLATFCDNILKKGGSEKLSDEAIEETLEKVVKLLAYISDKDLFAEFYRKKLARRLLFDKSANDEHERSILTKLKQQCGGQFTSKMEGMVTDLTLARENQASFEEYLSNNPAANPGIDLTVTVLTTGFWPSYKSFDLNLPAEMVRCVEVFKEFYQTKTKHRKLTWIYSLGTCNINGKFEPKTIELVVTTYQASALLLFNASDRLSYQEIMTQLNLSDDDVVRLLHSLSCAKYKILNKEPSTKTISPTDVFEFNFKFTDKMRRIKIPLPPVDEKKKVIEDVDKDRRYAIDASIVRIMKSRKVLGYQQLVMECVEQLGRMFKPDVKAIKKRIEDLITRDYLERDKDNPNLFKYLA

SEQ ID NO: 25 - protein, 738 aa, Brassica oleracea
MERKTIDLDQGWDYMQTGITKLKRILEGLPEPQFDSEQYMMLYTTIYNMCTQKPPHDYSQQLYDKYREAFEEYIHSTVLPALREKHDEYMLRELVKRWSNHKVMVRWLSRFFYYLDRYFIARRSLPPLNEVGLTCFRDLVYNELHSKVKDAVIALVDKEREGEQIDRALLKNVLDIYVEIGMGQMERYEEDFESFMLLDSASYYSRKASSWIQEDSCPDYMLKSEECLKKERERVAHYLHSSSEPKLVEKVQHELLVVYANQLLEKEHSGCRALLRDDKVDDLSRMYRLYHKIVKGLEPVANIFKQHVTAEGNALVQQAEDTATNHAANTASVQEQVLIRKVIELHDKYMVYVVECFQNHTLFHKALKEAFEIFCNKTVAGSSSAELLATFCDNILKKGGSEKLSDEAIEDTLEKVVKLLAYISDKDLFAEFYRKKLARRLLFDRSANDDHERSILTKLKQQCGGQFTSKMEGMVTDLTLARENQNSFEEYLGNNPAANPGIDLTVTVLTTGFWPSYKSFDINLPAEMVKCVEVFKGFYETKTKHRKLTWIYSLGTCHLNGKFDVKPIELVVSTYQAAVLLLFNTTDKLSYTDILTQLNLSHEDLVRLLHSLSCARYKILLKEPSTKTVSQSDSFEFNSKFTDRMRRIKIPLPPVDERKKVVEDVDKDRRYAIDAAIVRIMKSRKVLGHQQLVSECVEQLSRMFKPDIKAIKKRMEDLITRDYLERDKENANMFRYLA

SEQ ID NO: 26 - protein, 743 aa, Daucus carota
MMIERKTIDLEQGWDFMQKGITKLKNILEGFPEPQFSSEDYMMLYTTIYNMCTQKPPHDYSQQLYEKYREAIEEYITSTVLPSLREKHDEFMLRELVKRWSNHKVMVRWLSRFFHYLDRYFIARRSLPPLHEVGLTCFRDLVYQEINGKVRDAVISLINQEREGEQIDRALLKNVLDIFVEVGMSQMDYYENDFEADMLKDTAAYYSRKASNWILEDSCPDYMLKAEECLRREKDRVSNYLHSSSEPKLLEKVQHELLSHYATQLLEKEHSGCHALLRDDKVADLSRMYRLFSKIPRGLDPVSNIFKQHVTAEGTALVKQAEDAASNKKAEKRDVVGLQEQVFVRKIIELHDKYLTYVNDCFTNHTLFHKALKEAFEIFCNKGVSGSSSAELLATFCDNILKKGGSEKLSDEAIEETLEKVVRLLAYISDKDLFAEFYRKKLARRLLFDKSANDEHERSILTKLKQQCGGQFTSKMEGMVTDLTLAKENQSNFEEYLNNNSNVNPGIDLTVTVLTTGFWPSYKSFDLNLPAEMVKCVEVFREFYQTKTKHRKLTWIYSLGTCNIIGKFDPKTMELIVTTYQASALLLFNSSDRLSYNEIMTQLNLSDDDVVRLLHSLSCAKYKILSKEPNTKTISPTDCFQFNSKFTDKMRRIKIPLPPVDEKKKVIEDVDKDRRYAIDASIVRIMKSRKVLGYQQLVMECVEQLGRMFKPDVKAIKKRIEDLITRDYLERDKDNANLFRYLA

SEQ ID NO: 27 - protein, 742 aa, Apium graveolens
MNERKTIDLDNGWEFMQKGITKLKKILEGQPEPQFSSEDYMMLYTTIYNMCTQKPPHDYSQQLYDKYREAFEEYITSTVLPSLREKHDEFMLRELVNRWTNHKVMVRWLSRFFHYLDRYFIARRSLPALHEVGLTCFRDLVYQELKVKVRDAVISLIDQEREGEQIDRALLKNVLDIFVEIGMSQMDQYENDFEEAMLTDTAAYYSRKASNWILEDSCPDYMLKAEECLRREKDRVSHYLHFSSEPKLLEKVQHELLSVYATQLLEKEHSGCHALLRDDKVDDLSRMYRLFSKIPKGLDPVSYIFKQHVTNEGMALVKQAEDAASNKKAEKRDVVSLQEQVFVRKIIELHDKYLAYVNDCFTNHTLFHKALKEAFEIFCNKGVAGSSNAELLATFCDNILKKGGSEKLSDEAIEETLEKVVKLLAYISDKDLFAEFYRKKLARRLLFDKSANDEHERSILTKLKQQCGGQFTSKMEGMVTDLTLAKENQSSFEEYLGNNANVNPGIDLTVTVLTTGFWPSYKSFDLNLPAEMVKCVEVFREFYQTKTKHRKLTWIYSLGTCNINGKFEPKTIELIVTTYQASALLLFNTSDRLSYQEIMTQLNLSDDDVVRLLHSLSCAKYKILTKEPNNKTISPTDYFEFNSKFTDKMRRIKIPLPPVDEKKKVIEDVDKDRRYAIDASIVRIMKSRKVLGYQQLVMECVEQLGRMFKPDVKAIKKRIEDLITRDYLERDKDNANLFRYLA

SEQ ID NO: 28 - protein, 742 aa, Cichorium intybus
MNERKTIDLEQGWDFMQKGITKLKNILEGLPEPQFSSEDYMMLYTTIYNMCTQKPPHDYSQQLYDKYRESFEEYITSTVLPSLREKHDEFMLRELVRRWSNHKVMVRWLSRFFHYLDRYFIARRSLPPLNEVGLACFRDLVYQEVNGKVRDAVISLIDQEREGEQIDRALLKNVLDIFVEIGMGQMEYYENDFEASMLNDTAAYYSRKASNWILEDSCPDYMLKAEECLKREKDRVSHYLHSSSEPKLLEKVQTELLSVYATQLLEKEHSGCHALLRDDKVDDLSRMYRLFSKIQKGLDPVSSMFKQHVTAEGTTLVKQAEDAASTKKAEKRDVVGLQEQVFVRKVIELHDKYLAYVNDCFMNHTLFHKALKEAFEIFCNKGVAGSSSAELLATFCDNILKKGGSEKLSDEAIEDTLEKVVKLLAYISDKDLFAEFYRKKLARRLLFDKSANDEHERSILTKLKQQCGGQFTSKMEGMVTDLTLAKENQSHFEEYLNNNPNVSPGIDLTVTVLTTGFWPSYKSFDLNLPAEMVKCVEVFREFYQTKTKHRKLTWIYSLGTCNINGKFEPKTMELIVTTYQASALLLFNSSDRLSYQEIMTQLNLSDDDVVRLLHSLSCAKYKILLKEPNTKTISPTDFFEFNSKFTDKMRRIKIPLPPVDEKKKVIEDVDKDRRYAIDASIVRIMKSRKVLGYQQLVMECVEQLGRMFKPDVKAIKKRIEDLITRDYLERDKENPNLFRYLA

SEQ ID NO: 29 - protein, 742 aa, Cichorium endivia; identical to SEQ ID NO: 28

SEQ ID NO: 30 - protein, 744 aa, Allium ampeloprasum
MSLHERKTIDLEQGWAFMQKGITKLKNILDELNEPQFSSEDYMMLYTTIYNMCTQKPPHDYSQELYDKYRESFEEYITTTVLPSLREKHDEYMLRELVRRWSNHKIMVRWLSRFFHYLDRYFIARRSLPALNEVGLTCFRDLVYNEVHGKVKDAVISLIDQEREGEQIDRALLKNVLGIFVEIGLGSMECYENDFETSMLNATAAYYSRKASNWILEDSCPDYMLKAEECLKHEKDRVAHYLHSSSEQKLLEKVQHELLFVYASQLLEKEHSGCHALLRDDKVGDLSRMYRLFCRITRGLDPVSQIFKQHVTAEGTALVKHAEDAASNKKAEKKDIVGLQEQVFVRKVIELHDKYLAYVTDCFQNHSLFHKALKEAFEVFCNKGVAGSSSAELLAAFCDNILKKGGSEKLSDEAIEDTLEKVVKLLAYISDKDLFAEFYRKKLARRLLFDKSANDDHERSILTKLKQQCGGQFTSKMEGMVTDLTLARENQSSFDDYLSSNPKANSGIDLTVTVLTTGFWPSYKSFDLNLPDEMVKCVEIFKEFYETKTKHRKLTWIYSLGTCNINGKFETKTIELVVTTYQAAVLLLFNSADKLSYSEIVQQLNLSDDDVIRLLHSLSCAKYKILNKEPATKTITPNDHFEFNSKFTDRMRRIKIPLPPVDEKKKVIEDVDKDRRYAIDASIVRIMKSRKVLGHQQLVLECVEQLGRMFKPDFKAIKKRIEDLIARDYLERDKDNPNLFKYLA

SEQ ID NO: 31 - protein, 742 aa, Lactuca sativa
MNERKTIDLEQGWDFMQKGITKLKNILEGLPEPQFSSEDYMMLYTTIYNMCTQKPPHDYSQQLYDKYRESFEEYITSTVLPSLREKHDEFMLRELVRRWSNHKVMVRWLSRFFHYLDRYFIARRSLPPLNEVGLACFRDLVYQEVNGKVRDAVISLIDQEREGEQIDRALLKNVLDIFVEIGMGQMEYYENDFEASMLNDTAAYYSRKASNWILEDSCPDYMLKAEECLKREKDRVSHYLHSSSEPKLLEKVQNELLSVYATQLLEKEHSGCHALLRDDKVDDLSRMYRLFSKIPKGLDPVSSMFKQHVTAEGTTLVKQAEDAASTKKAEKRDVVGLQEQVFVRKVIELHDKYLAYVNDCFMNHTLFHKALKEAFEIFCNKGVAGSSSAELLATFCDNILKKGGSEKLSDEAIEDTLEKVVKLLAYISDKDLFAEFYRKKLARRLLFDKSANDEHERSILTKLKQQCGGQFTSKMEGMVTDLTLAKENQSHFEEYLNNNPNVSPGIDLTVTVLTTGFWPSYKSFDLNLPAEMVKCVEVFREFYQTKTKHRKLTWIYSLGTCNINGKFEPKTMELIVTTYQASALLLFNLSDRLSYQEIMTQLNLSDDDVVRLLHSLSCAKYKILLKEPNTKTISPTDYFEFNSKFTDKMRRIKIPLPPVDEKKKVIEDVDKDRRYAIDASIVRIMKSRKVLGYQQLVMECVEQLGRMFKPDVKAIKKRIEDLITRDYLERDKENPNLFRYLA

SEQ ID NO: 32 - protein, 738 aa, Raphanus sativus
MERKTIDLEQGWDYMQTGITKLKRILEGLPEPQFDSEQYMMLYTTIYNMCTQKPPHDYSQQLYDKYREAFEEYIDSTVLPALKEKHDEYMLRELVKRWSNHKVMVRWLSRFFYYLDRYFIARRSLPPLNEVGLTCFRDRVYKELHSKVKDAVIALVDKEREGEQIDRALLKNVLDIYVEIGMGQMERYEVDFESFMLLDSASYYSRKASNWIQEDSCPDYMLKSEECLKKERERVAHYLHSSSEPKLVEKVQHELLVVYANQLLEKEHSGCRALLRDDKVDDLSRMYRLYHKIAKGLEPVANIFKQHVTAEGNALVQQAEDTATNQAANTASVQEQVLIRKVIELHDKYMVYVVECFQNHTLFHKALKEAFEIFCNKTVAGSSSAELLATFCDNILKKGGSEKLSDEAIEDTLEKVVKLLAYISDKDLFAEFYRKKLARRLLFDRSANDDHERSILTKLKQQCGGQFTSKMEGMVTDLTLARENQTSFEEYLGNNPAANPGIDLTVTVLTTGFWPSYKSFDINLPSEMVKCVEVFKGFYETKTKHRKLTWIYSLGTCHLNGKFDHKPIELVVSTYQAAVLLLFNTTDKLSYNDILTQLNLSHEDLVRLLHSLSCARYKILLKEPSTKTVTQTDSFEFNAKFTDRMRRIKIPLPPVDERKKVVEDVDKDRRYAIDAAIVRIMKSRKVLGHQQLVSECVEQLSRMFKPDIKAIKKRMEDLITRDYLERDKENPNMFRYLA

SEQ ID NO: 33 - protein, 740 aa, Spinacia oleracea
MNDRKVIELEQGWEFMGKGITKLKRILEGLPEPPFNSEDYMMLYTTIYNMCTQKPPHDYSQQLYDNYKEAFVDYIHSTVLPSLGDKHDEFMLRELVKRWSNHKVMVRWLSRFFHYLDRYFIARRSLPSLNDVGLTCFRDLVYQEISGKAKDAVIALIDEEREGGQIDRALLKNVLDIYVEIGMTQMDYYEKDFEAHMLDDTAAYYSRKASSWILEDSCPEYMLKSEECLKKEKDRVAHYLHSSSEPKLLEKVQNELLLVYENQLLEKENSGCRALLKDDKVEDLSRMYRLYSKVTKGLEPIGSIFKQHITDEGTALVQQAEDAAISKAENAGGGSHEQVFVRKVIELHDKFMTYVTDCFNSHTIFHKALKEAFEVFLNKGVAGSSSAELLASFCDNILKKGGSEKLSDEAIEDSLEKVVKLLAYVSDKDLFAEFYRKKLSRRLLFDKSANDDHERSILTKLKQQCGGQFTSKMEGMVTDLTLARENQTNFEEYLGQNTDASPGLDLTVTVLTTGFWPSYKSSDLNLPAEMVRCVEVFKQFYQTKTKHRKLTWVYSLGSCNINGKFGPKTIELVVGTYQAAALMLFNTSDRLSYSEITTQLNLADEDLVRVLQSLSCAKYKILLKEPSTRNVISTDCFSFNSNFTDRMRRIRIPLPPMDERKKVVEDVDKDRRYAIDASIVRIMKSRKALGYQQLITECVEQLSRMFKPDFKAIKKRIEDLITRDYIERDKENPQLFRYLA

SEQ ID NO: 34 - protein, 739 aa, Beta vulgaris
MNDRKVIELEQGWEFMGKGITKLKRILEGLPEPPFNSEDYMMLYTTIYNMCTQKPPHDYSQQLYDNYKQAFVDYINSTVLPSLREKHDEFMLRELVKRWANHKVMVRWLSRFFHYLDRYFIARRSLPSLNEVGLTCFRDLVYQEISGKAKDAVIALIDIEREGGQIDRSLLKNVLDIYVEIGMGQMDHYEKDFEAHMLDDTAAYYSRKASSWILEDSCPEYMLKSEECLKKEKERVANYLHSSSEPKLLEKVQNELLLVYESQLLEKENSGCRALLKDDKVDDLSRMYRLYSKVTKGLEPIGSIFKQHITDEGTALVQQAEDAAISKAENTGGSHEQVFVRKVIELHDKFMTYVTDCFNSHTIFHKALKEAFEVFLNKGVAGSSSAELLATFCDNILKKGGSEKLSDEAIEDSLEKVVKLLAYVSDKDLFAEFYRKKLSRRLLFDKSANDDHERSILTKLKQQCGGQFTSKMEGMVTDLTLARENQTNFEEYLSQNPDASPGLDLTVTVLTTGFWPSYKSSDLNLPAEMVRCVEVFKQFYSTKTKHRKLTWVYSLGSCNINGKFGPKTIELVVGTYQAAALMLFNTSDRLSYSEIATQLNLADEDLVRVLQSLSCAKYKILLKEPNTKTVSPTDCFSFNSSFTDRMRRIRIPLPPMDERKKVVEDVDKDRRYAIDASIVRIMKSRKVLGYQQLITECVEQLSRMFKPDFKAIKKRIEDLITRDYIERDKENPQLFRYLA

SEQ ID NO: 35 - DNA, 2235 bp, Cucumis sativus
  source 1..2235: /organism="Cucumis sativus" /mol_type="unassigned DNA"
atgacaatgggcgagcggaagactattgacttggagcagggatgggagtttatgcagaagggtatcacaaagttgaagaacattctcgagggcttgcctgagcctcagttcagctccgaggactacatgatgctttacactaccatgtataacatgtgcacccaaaagccgccgcatgattactcccagcagctgtatgataaatatcgtgaatcttttgaagagtacatcacttctatggtcttaccatccttgagggagaagcacgatgagttcatgttgagagaactagtaaaaaggtggacaaaccataaagtcatggtgaggtggctttctcgcttcttccactatcttgatcggtacttcatcgctcgaaggtcacttccacctctaaatgaagttggcctcacatgcttccgcgaattggtgtacaaagagctaaatagtaaagtgagggatgcagtaatttcattgattgatcaagaacgtgaaggagaacagattgacagagctctactgaagaatgtactagatatatttgtggaaattggtatggggcaaatggattactatgaaaatgactttgaagctgccatgcttaaagatactgctgcttattactctaggaaggcttccaattggatcctagaagattcttgtcccgattatatgcttaaagcagaggagtgcttgaaacgagaaaaggatagggtttcccactatttgcactctagtagcgagccaaagttgttggagaaagttcaacatgaactattatctgtttatgctactcaactgctggaaaaagagcattcaggatgccatgcattgcttagagatgacaaggtggaagatttgtcaaggatgttccgtctattctccaaaataccgaagggactggatccagtttccaacatatttaagcagcatgtaactgctgaaggaacagcactggtcaaacaggcagaagatgctgcaagtaacaagaaggctgagaaaaaggacatagttggtctgcaggaacaggtttttgtaagaaaagtgattgagcttcacgacaagtacttggcttatgtgaatgattgtttccaaaaccacacacttttccataaggctctcaaggaagcttttgaagtattttgcaataagggtgttgctggaagttctagtgcagaattgcttgctaccttttgtgataacatccttaagaaaggtgggagtgagaagttgagtgatgaagcaatcgaggagacacttgagaaggttgtgaagttgttggcatacatttgcgacaaagatctgtttgctgaattctatagaaaaaaacttgcccgaaggcttctctttgacaagagcgcgaacgatgaccacgagagaagtatattgaccaaattgaagcaacaatgtggtggtcagttcacttctaagatggagggaatggttactgatttgactttggcaagggagaaccaaactagttttgaggagtatctgagcaataatccacaagcgagtcctggcatcgacctgactgttactgttttaactactggattttggccaagctacaagtcttttgacctcaacctgccggcagagatggtaaagtgtgttgaagttttcagagagttttatcaaacaaaaaccaagcatcgaaaacttacatggatttactcattgggtacttgtaacatcagtggaaaatttgaaccgaaaacgatggagctgattgtgacaacttatcaggcttctgccctgttgctattcaattcttcggatagactaagttactcggaaatcatgacacaattaaatttgagtgacgatgatgtagttagactactccactcgttgtcatgtgccaagtataaaattcttaataaggaaccaaatacgaaaaccatctctccgaacgatcattttgagttcaatgcaaaattctccgacaaaatgaggagaataaagatccctcttccgcctgtggatgagaaaaagaaagtcattgaagatgttgacaaggatcgaaggtatgctattgacgcctcaatcgtgcgtatcatgaagagtcggaaagttcttggtcatcagcaactagtgatggagtgcgtcgagcaattgggccgtatgttcaagcccgatttcaaggcgataaagaagagaattgaagacctgatcactcgggattatctagagagagacaaagacaacccccacttgtttaggtacttggcttga

SEQ ID NO: 36 - DNA, 2235 bp, Cucumis melo
  source 1..2235: /organism="Cucumis melo" /mol_type="unassigned DNA"
atgacaatgggcgagcggaagactattgacttggaacagggatgggagtttatgcagaagggtatcacaaagttgaagaacattcttgagggcttgcctgagccccagttcagctccgaggactacatgatgctttacactaccatgtataacatgtgcacccaaaagccgccgcatgattactcccagcagctgtatgataaatatcgtgaatcttttgaagagtacatcacttctatggtcttaccatccttgagggagaagcatgacgagttcatgttgagagaactagtcaaaaggtggacaaaccataaagtcatggtgaggtggctttctcgcttcttccactatcttgatcggtacttcatcgctcgaaggtcacttccacctctaaatgaagttggcctcacatgcttccgcgaattggtgtacaaagagctaaacagtaaagtgagggatgcagtaatctcattgattgatcaagaacgtgaaggagaacagattgacagagctctactgaagaatgtattagatatatttgtggaaattggtatggggcaaatggattactatgaaaatgactttgaagctgccatgcttaaagatactgctgcttattactctaggaaggcttccaattggatcctagaagattcttgtcccgattatatgctaaaagcagaggagtgcttgaagcgagaaaaggatagggtttcccactatttgcactctagtagcgagccaaagttgttggagaaagttcaacacgaactgttatctgtgtatgctactcaactgctggaaaaagagcattcaggatgccatgcattgcttagagatgacaaggtggaagatttgtcaaggatgttccgtctcttctccaaaataccgaagggattggacccagtttccaacatatttaagcagcatgtaactgctgaaggaacagcactggtcaaacaggcagaagatgctgcaagtaacaagaaggccgagaaaaaggacatagttggtctgcaggaacaggtttttgtaagaaaagtgattgagcttcacgacaagtacttggcttatgtgaatgattgtttccaaaaccacacacttttccataaggctctcaaggaagcttttgaagtcttttgcaataagggtgttgctggaagttctagtgcagaattgcttgctaccttctgcgataacatccttaagaaaggtgggagtgagaagttgagtgatgaagcaatcgaagagacacttgagaaggttgtgaagttgttggcatacatctgcgacaaagatctgtttgctgaattctatagaaaaaaacttgcccgaaggcttctctttgataagagcgccaacgatgaccacgagagaagtatattgaccaaattgaagcaacaatgtggtggtcagttcacttctaagatggagggaatggttactgatttgactttggcaagggagaaccaaactagtttcgaagagtatctgagcaataatccacaagctagtcctggaatcgacctaactgttactgttttgactactggattttggccaagctacaagtcttttgacctcaacctgccggcggagatggtaaagtgtgttgaagttttcagagagttttatcaaacaaaaaccaagcatagaaaacttacatggatttactcattgggtacttgtaacatcagtggaaaatttgaaccgaagacgatggagctgattgtgacaacatatcaggcttctgccctgttgctattcaattcttcggacagactaagttactccgaaatcatgacacaattaaatttgagtgatgatgatgttgttagactgctccactcattgtcgtgtgccaagtataaaattcttaataaggagccaaatacgaaaaccatctcaccgaacgatcattttgagttcaatgcaaaattctccgacaaaatgaggagaataaagatccctcttccgcctgtggatgagaaaaagaaagtcattgaagatgttgacaaggatcgaaggtatgctattgacgcctcaatcgtgcgtatcatgaagagtcgaaaagttcttggtcatcagcaactagtgatggagtgcgtcgagcaattgggtcgtatgttcaagcccgatttcaaggcgataaagaagagaattgaagacctgatcactcgggactatctagagagagacaaagacaacccccacttgtttaggtacttggcttga

SEQ ID NO: 37 - DNA, 2235 bp, Cucurbita pepo
  source 1..2235: /organism="Cucurbita pepo" /mol_type="unassigned DNA"
atgacaatgggtgagcggaagactattgacttggagcaaggatgggagtttatgcagaagggaatcacaaaattgaagaacattctggaaggattgcctgagccacagttcagctccgaggactacatgatgctttacactacaatgtataacatgtgtacccagaagccaccgcatgattactcccagcagctgtatgataaataccgcgaatcgtttgaggagtacatcagttctatggttttaccatccttgagggagaagcatgacgaatttatgttgagagaactggtcaaaaggtggaccaaccataaagtcatggtgaggtggctttctcgcttcttccactatcttgatcgatacttcattgctcgaaggtcacttccacctctcaatgaagttggcctcacttgcttccgtgaattggtgtacaaagagctaaacagtaaagtgagggatgcagtaatttcattgatcgatcaagaacgtgaaggagagcagattgacagagctctgttgaagaacgtgttggatatatttgtggagattgggatggggcaaatggattattatgaaaatgactttgaagctgccatgcttaaagatactgctgcttactactctaggaaggcatcaaattggatcttagaagattcttgtcctgattatatgctaaaagcagaggagtgcttgagacgagaaaaggaccgagtttctcactatctgcactctagtagcgagccaaagttattggagaaagttcaacatgaactattgtctgtttatgctactcaactgctggagaaagagcattcaggatgccatgcattgcttagagatgacaaggtggaagatttgtcaaggatgttccgtctcttctccaaaatacccaagggattggacccagtttccaacatatttaagcagcatgtcactgctgaaggaacagcattagtcaaacaggcagaagacgctgcaagtaacaagaaggccgagaaaaaggacatcgttggtctgcaagaacaggtttttgttagaaaagtgattgagcttcacgacaagtacttggcatatgtgaatgattgtttccaaaaccacacactttttcacaaggctctcaaggaagcttttgaagtcttttgcaataagggtgttgctggaagttctagtgcagaattacttgctaccttttgtgataacatccttaagaaaggtgggagtgagaagttgagtgatgaagcaattgaggaaacactcgagaaggtcgtgaaattgctggcgtatatctgcgacaaagatctgtttgctgaattctatagaaaaaaactcgcccgaaggcttctcttcgacaagagtgcgaatgatgaccacgagagaagtatactgacgaaattgaagcaacaatgtggtggtcagtttacctctaagatggagggaatggtcacggatttgacactggcaagggagaaccaaactagttttgaggaatatctgagcaataatccacaagctagtcctggaatcgacttgaccgttaccgttttgaccactggtttttggccaagctacaagtcttttgacctcaacctgccggcggagatggtaaagtgtgttgaagttttcagggaattttatcaaacaaaaaccaagcacagaaaacttacgtggatttactcgttgggtacctgtaacatcagcggaaaattcgaaccgaaaacgatggagctgatcgtgacaacctatcaggcttctgccctgctgcttttcaattcctcggataaactaagttactccgagatcatgactcaattaaacttgagtgacgatgatgttgttagactgctccactcgttgtcgtgtgcgaagtataaaattcttaacaaggagccaaatacgaaaaccatctctccgaacgatcattttgagttcaacgcaaaattctccgacaaaatgaggagaataaagatccctcttccgcctgtggatgagaaaaagaaagtaatagaagatgttgacaaggatcgaagatatgctatcgatgcctcgatcgtgcgtatcatgaagagtaggaaagttctgggtcaccagcagttagtgatggagtgcgtcgagcaactgggtcgtatgttcaagcctgatttcaaggcgataaagaagagaatcgaagatctgatcactcgtgactatttagagagagacaaagacaacccccacttgtttaggtacttggcttga

SEQ ID NO: 38 - DNA, 2235 bp, citrillus lanatus
  source 1..2235: /organism="citrillus lanatus" /mol_type="unassigned DNA"
atgacaatgggcgagcggaagactattgacttggaacaaggatgggagtttatgcagaagggaatcacaaagttgaagaacattcttgagggcttgcctgagcctcagttcagctccgaggactacatgatgctttataccaccatgtacaacatgtgcacacaaaagccgccacatgattactcccagcagctatacgataaataccgtgaatcttttgaggagtatatcacttctatggtcttaccatccttgagggagaagcatgacgagttcatgttgagagaactggtcaaaaggtggacgaaccataaagtcatggtgaggtggctttctcgcttcttccactatcttgaccgatacttcattgctcgaagatcacttccacctctcaacgaagttggcctcacatgcttccgtgaattggtgtacaaagagctaaacagtaaagtgagggatgcagtaatttcattgattgatcaagaacgtgaaggagagcagattgacagagctctactgaagaatgtattagatatatttgtggaaattgggatggggcaaatggattactatgaaaatgactttgaagctgccatgcttaaagatactgctgcttattactctaggaaggcttccaattggatcctagaagattcttgtcccgattatatgctaaaagcagaggagtgcttgaaacgagaaaaggatagagtttctcactatttgcactctagtagcgagccaaagttattagagaaagttcaacatgaactgttatctgtgtatgctactcaactgctggaaaaagagcattcaggatgccatgcattgcttagagatgacaaggtggaagatttgtcaaggatgttccgcctcttctccaaaatacccaagggattggacccagtttccaacatatttaagcagcatgtcactgctgaaggaacagcattggtcaaacaggcagaagatgctgcaagtaacaagaaggccgagaaaaaggacatagttggtctgcaggaacaggtttttgtaagaaaagtgattgagcttcacgacaagtacttggcttacgtgaatgattgtttccaaaaccacacactttttcacaaggctctcaaggaagcttttgaagtcttttgcaataagggtgttgctggaagttctagtgcagaattacttgctaccttttgtgataacatccttaagaaaggtgggagcgagaagttgagtgatgaagcaattgaggagacacttgagaaggtcgtgaagttgctggcatacatctgcgacaaagatctgtttgctgaattctatagaaaaaaacttgcccgaaggcttctctttgacaagagtgccaacgatgaccatgagagaagtatattgaccaaattgaagcaacaatgtggtggccagttcacctctaagatggaggggatggtcactgatttgactttggcaagggagaaccaaactagtttcgaggagtatctgagcaataatccacaagctagtcctggaatcgacttgactgtcactgttttgactactggcttttggccaagctacaagtcttttgacctcaacctgccggcagagatggtaaagtgtgttgaagttttcagagagttctatcaaacaaaaacaaagcatagaaaacttacatggatttactcattgggtacctgtaacatcagcggaaaatttgaaccgaaaacgatggagctgattgtaacaacttatcaggcttctgccctgctgctattcaattcctcagatagattaagttattccgagatcatgacacaattaaatttgagtgacgatgatgttgttagactgctccactcattgtcatgtgccaagtataaaattcttaataaggagccgaacacgaaaaccatctctccgaatgatcattttgagttcaatgcaaaattctccgacaaaatgaggagaataaagatccctcttccgcctgtggatgagaaaaagaaagtcattgaagatgttgacaaggatcgaaggtatgctattgatgcctcaatcgtgcgtatcatgaagagtcggaaagttctgggtcatcagcagctagtgatggagtgcgtcgagcaattgggtcgtatgttcaagcccgacttcaaagcgataaagaagagaatcgaagatctgatcactcgggactatttagagagagacaaagacaacccccacttgtttaggtacttggcttga

SEQ ID NO: 39 - DNA, 2229 bp, Solanum melongena
  source 1..2229: /organism="Solanum melongena" /mol_type="unassigned DNA"
atgaaccaacgcagcacaatcgatctggaacatggatgggatttcatgcaaaagggcatcacaaagctgaagaacattctagaagggctgcctgagcctcagttcagctcagaggactatatgatgctgtatacgacaatgtacaacatgtgtactcagaagcccccacatgattattctcaacagctgtatgacaaatatcgtgaagcttttgaagaatatatcacaacgacggtattaccttctttgagagaaaaacatgacgagttcatgttgcgagagttggtaaaaaggtggtcaaaccataaggtcatggttagatggttatcgcgattcttccattatcttgaccgttatttcattgctcggagatcactgccagggcttaatgaagttggactaacttgcttccgcgatctggtctaccaagagttgaatggaaaagtcagggatgctgttatatctctgattgatcaagagcgtgagggagagcaaattgacagagctctactgaagaatgtgctagatatatttgttgaaattggaatggggtcaatggattattatgagaatgattttgaagctgcaatgctcaaggacactgcggcttattattctcgcaaagcttctaactggatcctcgaagattcatgtccagattatatgctgaaagctgaggagtgcttgaaacgggagaaggatagggtctcccattatctccattctagcagtgagacaaagttgcttgagaaagtgcaacatgagttgttatctgtgtatgccaatcaacttcttgagaaggagcactctggatgccatgcattacttagagatgataaggtcgatgatttatcaaggatgtatagactcttttctaagattcctcgaggcttagagcctgtggctaatatatttaagcagcatgttactgctgaaggtacagctttggtgaaacaggctgaagatgctgctagcaacaaaaaggcagagaagagagatgtggttggtttgcaggaacaggtttttgttcggaaagtgattgagcttcatgataaatatttggcgtatgtgaataactgtttccaaaaccacacactttttcacaaggcacttaaagaagctttcgaacttttctgcaacaagggtgttgctggtagctcaaatgctgaacttcttgccacattctgcgacaacattctcaaaaaaggcgggagtgaaaaattgagtgatgaagccattgaagagacgctggagaaggtggtaaagctgctggcttatattagtgataaggacttgtttgcagaattctataggaaaaagctcgcccggcggttgttatttgataagagtgccaatgatgaacatgagagaagtatcctaacaaagttgaagcagcagtgtggaggtcagttcacatcaaagatggagggaatggtcacagatttgacattggcaagggaaaatcaagccagctttgaggagtatttgagcaataatccaacagcaaatccaggaattgacttgacggtgactgtcttgactactggcttctggcctagctacaagtcttttgatctcaacctcccagcagaaatggttaggtgtgttgaagtattcaaggagttttatcaaacaaaaacgaagcacaggaaacttacatggatatactctttgggaacttgcaacataaatggaaaatttgaggcaaagactattgagctcgttgtcactacttatcaggcttctgctctgcttctctttaatgcatcagatagattgagttatcaggaaatcatgacgcaattaaacctatcagatgatgatgttgttcggcttcttcattccctttcatgtgcgaaatacaagattctcaacaaggagccaagcaccaaaacaatttctccgactgatgtctttgagttcaactcaaagttcactgacaaaatgaggaggatcaagatacctctcccaccagttgatgaaaagaaaaaggtaattgaagacgttgacaaggataggcggtatgctatagatgcctcaattgtgcgtattatgaagagtcgtaaagtattgggctaccagcaactggtcatggagtgcgttgagcagttgggacgcatgttcaagcctgatgtcaaagctatcaagaagagaattgaagatctgataactagagattacctagagagggacaaagataacccaaacttgttcaagtacttggcatga

SEQ ID NO: 40 - DNA, 2229 bp, Solanum lycopersicum
  source 1..2229: /organism="Solanum lycopersicum" /mol_type="unassigned DNA"
atgaaccaacgaagcacaatcgatctggaacatggatgggacttcatgcaaaggggcattacaaagctgaagaacattctagaagggctgcctgagcctcaattcagctcagaggactatatgatgctatatacgacaatgtacaacatgtgtactcaaaagcccccacatgattattctcaacagctgtatgacaaatatcgtgaagcttttgaagaatatatcacaacaacggtattgccttctttgagagaaaaacatgacgagtttatgttgcgagagttggtaaaaaggtggtcaaatcataaagtcatggtcagatggttgtcaagattcttccattaccttgaccggtatttcattgcccggagatctctgccggggcttaatgaagttggactaacttgcttccgcgatcaggtctaccaagagttgaatggaaaagtcagggatgctgttatatctctgattgatcaagagcgtgagggagagcaaattgacagagctctacttaagaatgtgcttgatatatttgtcgaaattggaatggggttaatggattattatgagaatgattttgaagctgcaatgctcaaggacacagcggcttattattctcgcaaagcttctaattggatcctcgaagattcatgtccggattatatgctgaaagccgaggagtgcttgaaacgggagaaggatagggtctctcattatctccattcaagcagcgagacgaagttgcttgagaaagtgcaacatgagttgttgtctgtgtatgccactcaacttcttgagaaggagcactctggatgccatgcgttactgagagatgataaggttgaagatttatcaaggatgtataggctcttttctaagatttctcgaggcttagaccctgtggccaatatttttaagcagcatgttactgctgaaggtacagctttggtaaaacaggctgaagatgctgctagcaataaaaaggcagagaagagagatgtggttggtttgcaggaacaggtttttgttcggaaagtgattgaacttcatgataaatatttggcttatgtgaataactgtttccaaaaccacacactttttcacaaggcgcttaaagaagcttttgagcttttctgcaacaagggtgttgctggtagctcaagcgctgaacttcttgccaccttctgtgacaacattctcaaaaaaggcgggagtgagaaattgagtgatgaagctattgaagaaacgttggaaaaggtggtaaagctactagcttatattagtgataaggacttgtttgcagaattctataggaaaaagctagcccggcggttgttatttgataagagtgccaatgatgaacatgaaagaagtatcctaacaaagttgaagcagcagtgtggggggcagttcacatcaaagatggagggaatggtcacagatttgacattggcaagggaaaatcaagccagcttcgaggagtatttgagcaataatccaatagcaaatccaggaattgacttgacggtgactgtcttgactactggcttctggcctagctacaagtcttttgatctcaacctcccagcagaaatggttaggtgcgttgaagtatttaaggagttctatcaaacaaaaacaaagcacaggaaacttacgtggatatactctttgggaacttgcaacataaatggaaaatttgagccaaaaactattgagctcgttgtcactacttatcaggcttctgctctgctgctctttaatgcatcagatagattgagttatcaggaaatcatgacgcaattaaacctatcagatgatgatgttgttcggcttcttcattccctttcatgtgcgaagtacaagatactcaacaaggagccaagcaccaaaacaatttctccgactgatgtctttgagttcaactcaaagttcactgacaaaatgaggaggatcaagatacctctccctcctgttgatgagaagaaaaaggtaattgaagacgttgacaaggataggcggtatgctatagatgcttcaattgtgcgtattatgaagagccgtaaagtattgggctaccagcaactagtcatggagtgcgttgagcagttggggcgcatgttcaagcctgatgtcaaagctatcaagaagagaatcgaagatttgataactagagattacctagagagggacaaagataatccaaacctgttcaagtacttggcatga

SEQ ID NO: 41 - DNA, 2229 bp, Capsicum annuum
  source 1..2229: /organism="Capsicum annuum" /mol_type="unassigned DNA"
atgaaccagcgttccacaatcaatctagaacatggatgggacttcatgcaaaggggcattacaaagctgaagaacattctagaagggctgcccgagcctcagttcagctcagaggactatatgatgctgtatacgacaatgtacaacatgtgtactcagaagcccccacatgattattctcaacagctgtatgacaaatatcgtgaagcttttgaagaatatatcacaacaacggtattgccttctttgagagaaaaacatgacgagttcatgttgcgagagctggtaaaaaggtggtcaaaccataaggtcatggtcagatggttatcgcgattcttccattatcttgatcgctatttcattgcccggagatctctaccggggcttaatgaagttggactaacttgcttccgagatctggtctaccaagagttgaatggaaaagtcagggatgctgttatatctctgattgatcaagagcgtgagggagagcaaattgacagagctctactgaagaatgtgctagatatatttgttgaaattggaatggggtcgatggattattatgagaatgattttgaagctgcaatgctcaaggacaccgcagcttattattctcgcaaagcttctaactggatacttgaagattcatgtccagattatatgctgaaagccgaggagtgcttgaaacgggagaaagatagggtctctcactatcttcatttaagcagtgagacaaagttgcttgagaaagtgcaacatgagttgttgtctgtgtatgccactcaacttcttgagaaggagcactctgggtgccatgcgttactaagagatgataaggttgaagatttatcaaggatgtataggctcttttctaagattcctcgaggcttagaccctgtggctaatatatttaagcagcatgttactgctgaaggtacagctttggtcaaacaggctgaagatgctgctagcaacaaaaaggcagagaaaagagatgtggttggtttgcaggaacagatttttgttcggaaagtgattgagcttcatgataagtatatggcatatgtgaataactgtttccaaaaccacacactttttcacaaggcgcttaaagaagctttcgaacttttctgcaacaagggtgttgctggtagctcaagtgctgaacttcttgccacattctgcgacaatattctcaagaaaggcgggagtgagaaattgagtgatgaagccattgaagagacgctggagaaggttgtaaagctgctagcatatattagtgacaaggacttgtttgcagaattctataggaaaaagctagcccggcggttgttatttgataagagtgccaatgatgaacacgagagaagtatccttacaaagttgaagcagcagtgtgggggccagttcacatcaaagatggagggaatggtgacagatttgacattggcaagggaaaatcaagccagctttgaggagtatttgagcaacaatccagcagcaaatccaggaattgacttgacggtgactgtcttgactactggcttctggcctagctacaagtcttttgatctcaacctcccagcagaaatggttaggtgcgttgaagtattcaaggagttttatcaaacaaaaacgaagcacaggaaacttacgtggatatactctttgggaacttgcaatataaatggaaaatttgagccaaagactattgagctcgttgtcactacttatcaggcttctgctctgctgctctttaatgcatcggatagattgagttatcaggaaatcatgacgcaactaaacctatcagatgatgatgttgttcggcttcttcattccctttcatgtgcgaagtacaagattctcaacaaggagccaagcaccaaaacaatttctccgactgatgtctttgagttcaattttaagttcactgacaaaatgaggaggatcaagatacctctccctcctgttgatgagaagaaaaaggtaattgaagatgttgacaaagataggcggtacgctatagatgcttcaattgtgcgtattatgaagagtcgtaaagtattgggctaccagcaactggtcatggagtgtgttgagcagttgggacgtatgttcaagcctgatgtcaaagctatcaagaagagaattgaagatttgataactagagattacctagagagggacaaagataatccgaacttgttcaagtacttggcatga

SEQ ID NO: 42 - DNA, 2217 bp, Brassica oleracea
  source 1..2217: /organism="Brassica oleracea" /mol_type="unassigned DNA"
atggagcgcaagacgattgacttggaccaaggatgggactatatgcagactggtatcactaagctgaaacggattcttgaggggctgcctgagccgcagtttgactctgagcaatacatgatgctctatacgactatgtacaacatgtgcactcagaaacctcctcatgattactcacagcagctttatgacaagtatcgtgaagcatttgaggagtatattcactcaactgttttgcctgctctaagggagaagcatgatgagtacatgctgagggagctggttaagagatggtctaaccataaagttatggttcgatggctatcccgcttcttctactatcttgaccgttacttcattgctcggaggtcacttccacccctgaatgaagttggcctgacttgcttccgtgacctggtttataacgagttgcattccaaggtcaaagatgctgtaatagcacttgttgataaagaacgggagggtgagcagattgacagggctctattgaaaaacgtattagacatttatgtagagattggaatgggacagatggaaagatacgaggaggattttgaaagcttcatgcttttagattcagcatcttactattctcgcaaggcgtcaagctggatccaagaagattcttgccctgattacatgctgaagtctgaagaatgtcttaagaaggagagggagagagtggctcactaccttcactcaagcagcgagccaaagctggttgagaaagtacaacatgagctgttggtagtgtatgcaaatcagcttctagaaaaagagcattcagggtgccgtgcattgctgagagatgacaaggttgatgacctctccaggatgtacaggctttatcataaaattgtgaaaggtttggaacctgttgcaaacatatttaagcagcatgtcacagcagagggtaacgcacttgtccaacaggccgaagacacggccactaatcatgctgcaaatactgctagcgtgcaggaacaggttcttatcagaaaagtgattgaactacatgataaatacatggtctatgttgttgagtgtttccagaaccacaccctcttccacaaggcattgaaagaggcatttgagatattctgtaacaaaacagtcgctggaagttctagtgctgaattgcttgcaacattttgcgacaatattctcaagaaggggggaagtgaaaagctgagcgatgaagctattgaagatacccttgagaaggtggtcaaattgcttgcttatataagtgacaaggatcttttcgccgagttctacaggaagaagctggcccgtaggctcttatttgatcgcagtgctaatgatgatcatgagagaagtatcctgacaaagctcaagcaacaatgtggtgggcagtttacttcgaagatggagggcatggtgactgatttgacattggcaagggaaaaccaaaacagcttcgaggagtatcttggcaataaccccgctgcaaacccagggattgatttgaccgtaactgttcttaccactggtttttggccaagttacaaatcatttgacataaatctacccgctgaaatggtcaagtgtgttgaagttttcaaagggttttatgaaacaaagacaaaacataggaaacttacctggatctactcactaggaacttgccacctcaatgggaagtttgatgtcaagcccattgagttagttgtgtctacataccaggctgctgtgcttctgctgttcaacacaacagacaaattgagctacactgatatcctaactcagctgaacctgagccacgaagatctagtgaggttgcttcattccttgtcatgtgctagatacaagattcttctcaaggagccaagcacaaagactgtttcccagtctgattcttttgaattcaactccaaattcaccgacagaatgcggagaataaagatccctctcccacctgttgatgagaggaagaaagttgtggaagacgtggacaaagacagacgctatgcgattgatgctgccattgtgaggatcatgaagagcaggaaagtattgggacatcaacaacttgtttctgagtgcgttgagcaacttagccgaatgttcaagcctgatatcaaggcaatcaagaagcgcatggaggatttgataacgagagattatctggagagggacaaggagaacgctaacatgtttaggtacttggcttag

SEQ ID NO: 43 - DNA, 2232 bp, Daucus carota
  source 1..2232: /organism="Daucus carota" /mol_type="unassigned DNA"
atgatgattgagcggaaaactatagacctggagcagggatgggactttatgcaaaagggaatcacaaagctaaagaatattttagaaggctttccggagccgcaattcagctcggaggattatatgatgctttatacaactatgtataacatgtgtacacagaaacctccacatgattactctcagcagctgtatgaaaagtatcgtgaagctattgaggagtacattacttctacagtattgccttcattgagagagaagcatgatgaattcatgcttagagaacttgtgaagagatggtctaatcataaggtcatggtcaggtggctttctcgattctttcactatcttgatcgctattttattgctcggaggtcacttccaccacttcatgaagttggactcacttgctttcgggacctggtttaccaggagataaatgggaaagtaagggatgctgtaatatcattgattaatcaagagcgcgagggagagcaaattgaccgagctttgttgaagaatgttctagatatatttgttgaagttggaatgagtcaaatggattattatgagaatgactttgaagcagacatgctcaaagatacagcagcatactattctcgaaaggcttccaactggatcttagaagattcttgtccagattatatgctcaaagcggaagagtgtttgagacgggaaaaggacagggtctctaactaccttcattctagtagtgaacccaagttgcttgagaaagttcaacatgagttactatcacactatgcaactcagctgcttgagaaagaacactctgggtgtcatgcattgcttagggatgacaaggtggcagatttatcaaggatgtataggctcttctctaaaatacctcgaggcctagatcccgtgtctaatattttcaagcagcatgttactgctgaaggtacagctttggtcaaacaagcagaagatgcagctagcaacaagaaggcagagaagagagatgtagtaggtttacaagaacaggtttttgtgaggaaaataattgaattgcatgacaaataccttacatacgtaaatgactgttttacaaaccacactctcttccataaggcgcttaaggaggcttttgaaatcttctgcaataagggtgtctctggaagctctagtgcagaattacttgccacattctgtgataatattctcaagaaaggtggaagcgagaagttaagtgatgaagccattgaggaaacacttgagaaggttgtaaggttgcttgcttatataagtgacaaagacttatttgctgaattttataggaaaaagcttgcacggcgtctcttattcgacaagagtgccaatgatgagcatgagagaagtatattgactaagctgaagcaacaatgtgggggtcaatttacatcaaagatggaaggaatggtcactgacttgacgttggcaaaggaaaatcagtccaacttcgaggagtacctcaataataattcaaacgtaaatcctggaattgacttgacagttactgttctaaccactgggttttggccaagttacaaatctttcgatctcaacctcccagcagagatggtcaaatgtgttgaagtttttagagaattctaccaaacaaaaacaaagcacagaaaactgacatggatatactctttgggtacttgtaacatcattggaaaatttgatccaaaaaccatggagcttattgtgacaacataccaggcctctgctctgctgctatttaactcttctgatagacttagttataatgaaataatgactcagttgaacttgtcggatgatgatgttgtcagactacttcattctctttcgtgtgcaaagtacaagattctatctaaagagccgaacaccaaaactatatctccaactgattgctttcagttcaattccaaatttactgataaaatgaggaggattaagattccacttcccccagtggatgagaagaaaaaggtaattgaagatgttgataaagacaggcgatatgctatagatgcttcaattgtccgtatcatgaagagccgcaaagttttgggttatcagcagctagtaatggagtgcgttgaacaattgggtcgcatgtttaagcctgatgtcaaagcaatcaagaagagaatcgaagatttaataactcgggattatctggaaagagacaaggacaatgccaacttgttcaggtatctggcatga

SEQ ID NO: 44 - DNA, 2229 bp, Apium graveolens
  source 1..2229: /organism="Apium graveolens" /mol_type="unassigned DNA"
atgaacgagcggaagactatcgatttggataatggatgggaatttatgcagaaagggatcactaagttgaagaagattctcgaaggtcaacctgagcctcagtttagctccgaggactatatgatgctttacacaactatgtataatatgtgtacgcagaagcctccacatgattattctcaacagctgtatgacaagtaccgtgaggcctttgaggagtacataacttcaactgtcctgccttctttacgagagaagcatgatgagtttatgttgagagagctcgtgaatagatggacaaaccataaagtcatggtcaggtggctttctcgattctttcactatcttgatcggtacttcattgcgaggaggtcacttcctgcacttcatgaagttggactcacgtgcttccgggatctggtctatcaggagctgaaagttaaagtgagggatgctgtaatatctctgatcgatcaagagcgtgagggggaacagattgaccgagctttattaaagaacgtgttagatatatttgttgaaatcggaatgagtcaaatggatcaatatgagaatgactttgaagaagccatgctcactgatactgctgcttactattctcgaaaagcttcaaactggatccttgaagattcttgtcctgattatatgttaaaggcagaagaatgtttgcgacgagagaaggacagggtttcccactacctacattttagtagcgagccaaagttgcttgagaaagtgcaacatgagctgctatctgtgtatgcaacccaattactcgagaaggaacattctggttgtcatgcattgcttagggatgacaaggtggatgatttgtctaggatgtacagactcttctcgaaaatacctaaaggcctggatccagtttcttatatttttaagcagcatgttacaaatgaagggatggcattggttaaacaagcagaagatgcagcaagcaacaagaaggcagaaaagagagacgtggttagtttacaggagcaggtttttgttagaaaaattattgaattacatgacaaatacctcgcctatgtgaatgactgctttacaaaccatactcttttccataaggctctcaaggaggcttttgaaatcttttgcaacaagggtgttgctggaagctctaatgctgaactacttgctactttctgtgataacatcctcaaaaagggtgggagtgagaaattaagtgatgaggctattgaagaaacacttgagaaggtagtaaaattgttagcttacattagcgataaagacttgttcgctgaattttacagaaaaaagcttgcacggagacttctctttgataagagtgcaaatgacgagcatgaacgaagtattttgactaaactaaagcaacagtgcggtggtcagttcacatcgaaaatggaggggatggtcacagatttgactttggctaaagaaaatcaatccagctttgaggagtatctgggaaataatgccaatgtgaatcctggcattgacttgacggttactgttctgaccactggcttctggcctagttataaatcctttgatctcaaccttcctgctgagatggtcaagtgcgttgaagtatttagagaattttatcaaacaaaaacgaagcatagaaagctcacatggatatattctctgggtacttgtaatatcaatggaaaatttgaacccaaaaccattgagctgattgtgacaacctaccaggcctctgctctcctgttatttaatacttctgataggttgagttatcaagaaatcatgactcagttaaatttgtcggatgatgatgttgttcgcctgcttcattccctttcatgtgccaagtataaaattcttactaaagagccgaacaacaaaacaatttcccctacggattactttgagttcaactccaagttcactgacaaaatgaggagaattaagattccactacctccagttgatgagaagaaaaaggtaattgaagatgttgacaaggaccggcgatatgccattgatgcatctattgtccgcattatgaagagccgtaaagttttgggctaccaacaattggttatggaatgtgttgagcaattgggacgcatgtttaagcctgatgtcaaagcaattaagaagagaatcgaagatttaataacgcgtgattatctggaaagagacaaggataatgccaaccttttcagatatttggcatga

SEQ ID NO: 45 - DNA, 2229 bp, Cichorium intybus
  source 1..2229: /organism="Cichorium intybus" /mol_type="unassigned DNA"
atgaatgaaagaaaaacaatagacttagaacaaggatgggacttcatgcagaaaggcataacaaagttgaagaacattctagaaggtcttcccgagccacaattcagctcggaagattacatgatgctctacacaaccatgtacaatatgtgcacacaaaaaccgccacatgattactctcaacaattgtatgacaaataccgcgagtcttttgaagagtacattacttcaacggtgttaccttctttaagagagaagcatgatgagtttatgcttagagagcttgttagaagatggtcaaatcataaagtgatggttaggtggctttctagattcttccattatcttgatcgatacttcattgcccgaagatctcttccaccattaaatgaagttggacttgcgtgttttcgtgatctggtataccaagaggtgaatgggaaagtgagagatgctgtaatatctttgattgatcaagagcgtgaaggcgagcaaattgaccgagcattactcaagaatgttctagatatatttgttgaaataggaatgggacaaatggaatattatgagaatgattttgaagcatccatgcttaatgatacagcagcatattattcacgcaaagcttccaattggattctagaagattcttgtccagattatatgctcaaagctgaggagtgcttaaaaagagaaaaggacagagtttctcattatcttcattccagcagtgaaccaaagcttcttgagaaagttcaaacagagttattatctgtttatgcaactcaattgcttgaaaaggagcactccggttgtcatgcattacttagggatgacaaggttgatgatttatcaagaatgtacagactcttttcaaagatacaaaaagggctggatcctgtttctagtatgtttaagcagcatgtcactgctgaaggcacaacattggttaaacaggcagaagatgcagcaagtactaagaaggctgaaaagagagacgtggttggcttacaagaacaggtttttgttagaaaagttatcgagcttcatgacaagtaccttgcatatgtaaatgactgttttatgaatcataccctgtttcacaaggctcttaaagaggcatttgaaatattctgcaacaagggcgttgctggaagttcaagtgcagaattacttgctacattttgtgataatattcttaaaaaaggtggaagtgaaaaattgagtgatgaagccattgaggacacacttgagaaggtggtaaagttgcttgcttacatcagcgataaagatctatttgcagagttttataggaaaaaactggctagacggcttttatttgacaaaagtgcaaatgatgagcacgaaagaagtattttgacaaaattgaaacaacaatgtggcggtcaatttacatcaaaaatggaaggaatggttacagatttgacattggcaaaagaaaatcaatcacattttgaggagtatttgaataataatcccaatgttagccctggcattgacttgaccgtgactgtgttgaccactggtttttggcctagttacaaatcttttgacctaaatctccctgcagaaatggtcaaatgcgttgaagttttcagagaattttatcaaacaaaaacaaaacacagaaaactcacatggatatattcattgggcacctgcaatataaacggaaaattcgaaccaaaaaccatggagctaatcgttacaacttaccaggcatctgctttattactgttcaactcatcagatcgattgagttatcaagaaatcatgactcaattaaacttatcagatgatgatgttgttagactactccattcattatcatgtgcaaaatataaaattttattaaaagaaccaaatacaaaaacaatctctccaactgatttctttgaattcaactcaaagtttacagataaaatgagaaggatcaagattcctctacctcctgttgatgaaaagaaaaaagtaattgaagatgttgacaaagaccgacgttatgcaattgatgcttcaattgtacggataatgaaaagcagaaaagttcttggataccaacaattggtcatggaatgtgttgaacaattaggccgtatgtttaagcctgatgtaaaagcaatcaagaaacgtattgaagatctcataactcgtgattatcttgaaagagacaaagaaaatccaaatttgtttcggtacttggcatga

SEQ ID NO: 46 - DNA, 2229 bp, Cichorium endivia
  source 1..2229: /organism="Cichorium endivia" /mol_type="unassigned DNA"
atgaatgaaagaaaaacaatagacttagaacaaggatgggacttcatgcaaaaaggcataacaaagttgaagaacattctagaaggtcttcccgagccacaattcagctcagaggattacatgatgctctacacaaccatgtacaatatgtgcacacaaaaaccgccacatgattactctcaacaattatatgacaaataccgcgagtcttttgaagagtacataacttcaacggtgttaccttctttaagagagaagcatgatgagtttatgcttagagagcttgttagaaggtggtcaaatcataaagtgatggttaggtggctttctagattcttccattatcttgatcgatactttattgcaagaagatctcttccaccattaaatgaagttggacttgcgtgttttcgtgatctggtataccaagaggtgaatggaaaagtgagagatgctgtaatatctttgattgatcaagagcgtgaaggcgagcaaattgaccgagcattactgaagaatgttctagatatatttgttgaaataggaatgggacaaatggaatattatgagaatgattttgaagcatctatgcttaatgatacagcagcatattattcacgcaaagcttccaactggattctagaagattcttgtccagattatatgctcaaagctgaggagtgcttaaaaagagaaaaggacagagtttctcattatcttcattcaagtagtgaaccaaagcttcttgagaaagttcaaacagagttattatctgtttatgcaactcaattgctcgaaaaggaacactcaggttgtcatgcattacttagagatgacaaggttgatgatttatcaagaatgtacagactcttttcaaagatacaaaaaggactggatcctgtttccagtatgtttaagcagcatgtcactgctgaaggcacaacattagtaaaacaagcagaagatgcagcaagtactaagaaggctgaaaagagagacgtggttggcttacaggaacaggtttttgttagaaaagtaatcgagcttcatgacaagtacctcgcatatgtaaacgactgttttatgaatcacacattgttccacaaggctcttaaagaggcatttgaaatattctgcaacaagggcgttgctggaagttcaagtgcagaattacttgccacattttgtgataatattcttaaaaaaggtggaagtgaaaaattgagtgatgaagccattgaagacacacttgagaaggtagtaaagttgcttgcttacatcagcgataaagatctatttgcagagttttataggaaaaaactggctagaaggcttttatttgacaaaagtgcaaatgatgagcatgaaagaagtattttaacaaagttgaagcaacaatgtggtggtcagtttacatcaaagatggaaggaatggttacagatttaacactggcaaaagaaaatcaatcacattttgaggagtatttgaataataatcccaatgttagccctggcattgacttgaccgtgactgtgttgaccacgggattttggcctagttacaaatcttttgacctaaatcttcctgcagaaatggtcaaatgcgttgaagttttcagagaattttatcaaacaaaaacaaaacacagaaaactcacatggatttattcattgggcacctgcaatattaacggaaaattcgaaccaaaaaccatggagctaatcgttacaacttaccaggcatctgctttattgttattcaactcatcagatcgattaagttatcaagaaatcatgactcaattaaatttatcagatgatgatgttgttagactactacattcattatcatgtgcaaaatataaaattttattaaaagaaccaaataccaaaacaatatctccaaccgatttctttgaattcaactcaaagtttacagataaaatgagaaggatcaagattcctctacctcctgttgatgaaaagaaaaaagtaattgaagatgttgacaaagatagaaggtatgcaattgatgcttcaattgtacgaataatgaaaagcagaaaagttcttggataccaacaattggttatggagtgtgttgaacaattaggccgtatgtttaagcctgatgtaaaagcaatcaagaagcgtattgaagatttgataacgcgtgattatcttgaaagagacaaagaaaatccaaatttgtttcggtacttggcatga

SEQ ID NO: 47 - DNA, 2235 bp, Allium ampeloprasum
  source 1..2235: /organism="Allium ampeloprasum" /mol_type="unassigned DNA"
atgtcgttgcacgaaaggaaaaccattgatttggagcagggatgggcttttatgcagaaagggatcaccaaactgaagaatattcttgatgagttgaatgaacctcagttcagctcagaggattacatgatgctctatacgactatgtataatatgtgtactcagaagccgccacatgattattctcaggagttgtatgataagtaccgagagtcctttgaagagtatatcactaccactgtgcttccttcattgagagaaaagcatgatgaatacatgttaagggagctcgtgagaaggtggtcaaatcataaaataatggttagatggctttcacgctttttccattatcttgatcgctactttatagcacgaagatcattgcctgctcttaatgaagtcggtctcacttgtttccgtgatctggtgtacaacgaagtccatgggaaagttaaagatgccgtgatctcattgattgaccaagagagggaaggggagcaaattgacagagctttattaaagaatgttttgggtatttttgtagagattggtttgggaagcatggaatgttatgagaatgattttgaaacatcaatgcttaatgctacagcagcctattattcacgaaaagcttcaaattggattctagaagattcatgtccagattatatgctaaaagccgaggagtgcttaaaacatgagaaagatagagttgctcattatttgcattcaagcagtgaacagaagctgttagagaaagtgcaacatgagttacttttcgtatatgcaagtcaacttctcgagaaagaacattccggatgtcatgcattgcttcgcgatgacaaggtgggagatctttcacgcatgtatcggctgttctgtagaattacacgtggtttggaccctgtgtctcaaatatttaagcagcatgtgactgcagaaggtactgctttggtcaaacatgccgaagatgctgcaagtaacaagaaggccgagaaaaaagacattgttggtttgcaagagcaggtcttcgttaggaaagtaattgagctgcatgataaatacttggcctatgtgactgactgctttcaaaatcactctctatttcacaaggcacttaaagaggcattcgaggtattctgcaataaaggtgttgcaggtagctcaagcgctgaacttctggctgctttttgtgacaatatattgaagaagggtggaagcgagaaactaagcgatgaggccatagaggatactcttgagaaggttgtaaaactattggcatatattagcgataaagatctgtttgctgaattttacaggaagaagcttgcacgaagattactctttgacaaaagtgctaatgatgaccatgagaggagcatccttacaaagctgaaacagcaatgtggagggcagttcacctctaaaatggaaggcatggtaaccgatctgacacttgcacgagaaaatcaatcaagttttgacgattaccttagcagcaatcctaaagcaaattctggaattgacttgactgttacagtcttaacaactggcttctggcccagttacaagtcttttgatctcaatcttcctgatgagatggtaaaatgcgttgaaatttttaaagagttttacgagacaaaaaccaaacacagaaaacttacatggatttattcgttgggcacttgcaacatcaatggcaagttcgaaaccaagacaatagagttggttgttacaacctatcaggctgcagtgttgcttctattcaactctgcagataaattaagttattctgagattgtgcagcagctaaacttatctgatgatgatgtaatcagattacttcactctctttcatgcgctaaatacaaaattctcaataaagaacccgctaccaagactattaccccgaatgatcattttgagttcaattctaaattcactgatagaatgagaaggatcaagattcccctgcctcctgtggatgagaagaaaaaagtaattgaagatgttgacaaagacagaagatatgcaattgacgcatccatagttcgaataatgaaaagtagaaaagttcttggtcatcagcagcttgttttggaatgtgttgagcaattaggccgcatgtttaagcctgactttaaggccatcaagaaaaggattgaagatctgatcgctagagattatttggagagggacaaggacaatccaaacctctttaaatatttggcctaa

SEQ ID NO: 48 - DNA, 2229 bp, Lactuca sativa
  source 1..2229: /organism="Lactuca sativa" /mol_type="unassigned DNA"
atgaacgaaagaaaaacaatagacttagagcaaggatgggacttcatgcagaaaggaataacaaagttgaagaatattctagaaggtcttcccgagccacaattcagctcggaggattacatgatgctctacacaaccatgtacaacatgtgtacacagaaaccaccacatgattactcccaacagttgtatgacaaatatcgtgagtcttttgaagagtatattacttcaactgtgttaccttctttaagagagaagcatgatgagttcatgctgagagagcttgttagaaggtggtcaaatcataaagtcatggtgcggtggctttctagattcttccattatcttgaccgatatttcattgcccgaagatctcttccgccactaaatgaagttggacttgcctgttttcgtgatctggtataccaagaggtgaatggtaaagtgagagatgctgtaatatctttgattgatcaagagcgtgaaggggagcagattgatcgagctttactgaagaatgttctagatatatttgttgagataggaatgggacaaatggagtattatgagaatgattttgaagcatccatgcttaatgatacagcagcatattattcacgcaaggcttccaactggattctagaagattcttgtccagattatatgctcaaagcagaggagtgcttaaaaagagaaaaggacagagtgtctcattatcttcattccagcagtgagccaaagcttcttgagaaagttcaaaatgagttattgtctgtttatgcaactcaattgcttgagaaagagcactcaggttgtcatgcattgctcagggatgacaaggttgatgatttatcaagaatgtacagactcttttcaaagataccaaaaggattggatcctgtttctagtatgtttaagcagcatgtcactgctgaaggcacaacattggttaaacaagcagaagatgcagcaagtaccaagaaggctgaaaagagagatgtggttgggttgcaggaacaggtttttgttagaaaagttattgagctccatgacaagtacctggcatatgtaaatgactgtttcatgaaccatactcttttccacaaggctcttaaagaggcatttgaaatattctgcaacaagggtgttgctggaagttcaagtgcagagttacttgccacattttgtgataatattcttaaaaaaggtggaagtgagaaactgagcgatgaagccattgaggacacccttgagaaggtagtaaagttgcttgcctacatcagtgataaagatctatttgctgaattttacaggaaaaaacttgctaggaggcttttgtttgacaagagtgcaaacgatgagcatgagagaagtattctcacaaagctgaagcaacagtgtggtggtcagttcacatcaaagatggaagggatggttacagatttgacattggcaaaggaaaaccaatcccattttgaagagtatttgaacaataatcccaatgtcagccctggaattgacttgactgtcactgtgttgactaccggcttctggcccagctacaaatcttttgacctaaatctccctgccgaaatggttaaatgcgttgaagttttcagagaattttatcaaacaaaaacaaagcacaggaagcttacatggatatattcattgggtacctgcaatataaacgggaaatttgaacccaaaacaatggagctcatagtcacaacctaccaggcatctgctttattactgttcaacttatcggatcgattgagttatcaagaaatcatgactcagttgaacttgtcagatgatgatgttgttaggctgctccattctttgtcatgtgcaaaatacaaaattcttttaaaggagcctaataccaaaacaatctctccaaccgattacttcgaattcaactccaagtttacagataaaatgaggaggatcaagattcctctacctcctgtggatgagaagaaaaaggtgattgaggatgttgacaaagacagacgttatgccattgatgcttccattgtaaggataatgaagagcagaaaggtgcttggataccagcagttggttatggagtgtgttgaacagttgggacgcatgtttaagcctgatgtaaaagcaatcaagaagcggattgaagatctgataactcgtgattatcttgaaagagacaaagagaaccccaacttgttccgatacttggcatga

SEQ ID NO: 49 - DNA, 2217 bp, Raphanus sativus
  source 1..2217: /organism="Raphanus sativus" /mol_type="unassigned DNA"
atggagcggaagacgattgatctggaacaaggatgggactatatgcagactgggatcactaagctgaaacggattcttgaaggattgcctgagccgcaattcgactctgagcagtacatgatgctttatacgactatgtacaacatgtgcacccagaaacctcctcatgattactctcagcagctttatgacaagtatcgcgaagcttttgaggagtacattgactctactgttttgcctgctttgaaggagaagcatgatgaatacatgctacgggagctggttaagagatggtctaaccataaagttatggttagatggctatcccgattcttctactatcttgaccgttacttcattgctcggagatcgctgccaccgcttaatgaagttgggctcacatgcttccgtgaccgggtgtataaggagttgcattccaaggtcaaagatgctgtaatagcacttgttgataaagaacgggaaggcgagcagattgacagggctcttctgaaaaacgtattagatatctatgtagagattggaatgggacagatggaaagatacgaagtggattttgaaagcttcatgcttttggattcagcatcttactattctcgcaaagcatcaaactggatccaggaagattcttgccctgattacatgctgaagtctgaagaatgccttaagaaggagagggagagggttgctcactaccttcattcaagcagcgagccaaagctggttgagaaagtacaacatgagctgttggttgtctatgcaaatcagcttcttgaaaaggagcactcagggtgccgtgcattgctgagagacgacaaggttgacgatctctccaggatgtacaggctctatcataaaattgctaaaggtttagaacctgttgcaaacatatttaagcagcatgtcacagccgagggtaacgcacttgtccaacaggccgaagacacagccactaatcaggctgcaaatactgctagcgtgcaggaacaggttctcatcagaaaagtgattgagctacatgataagtacatggtctatgtcgtggagtgcttccagaaccacaccctcttccacaaggctctgaaagaggcatttgagatattctgtaacaaaacagtcgctggaagttcaagtgcagaactgcttgcaacattctgcgacaacatcctcaagaaggggggtagtgagaagctgagtgacgaagctattgaagatacgcttgagaaggttgtcaaattgcttgcttatataagcgacaaggatcttttcgccgagttctacaggaagaagctggcacgtaggctcttatttgatcgcagtgcgaatgatgatcatgagagaagcatccttacaaagctcaagcaacaatgtggtgggcagttcacttctaagatggagggcatggtaacggacttgacattggcaagagagaaccaaaccagtttcgaggagtatctaggcaataaccccgctgcaaacccagggattgatttgaccgtcactgttcttaccactggtttctggccaagttacaaatcattcgacataaatctaccaagtgaaatggtcaagtgtgttgaagttttcaaagggttttatgagacgaaaactaaacataggaaacttacatggatctactcactaggaacttgtcacctcaacggaaagtttgatcacaagcccattgagttagttgtgtctacttaccaggctgctgtgcttctgctgttcaacacaacagacaaattgagctacaacgatatcctaactcaactgaacctaagccacgaagatttagtgaggttgcttcattccctgtcatgtgctaggtacaagatccttctcaaggagccaagcacgaagactgttacacagactgattcatttgaattcaatgccaaattcacggacagaatgcgcagaatcaagatccctctccctcctgttgatgaaaggaagaaggttgtggaagatgtggacaaagacagacgctatgcgattgatgctgccattgttaggatcatgaagagcaggaaagtgttgggacatcaacaactcgtctctgagtgcgttgagcaacttagccgaatgttcaagcctgatatcaaagcgatcaagaagcgtatggaggatctaattacgagggattatttggagagggacaaggagaaccctaacatgtttaggtacttggcttag

SEQ ID NO: 50 - DNA, 2223 bp, Spinacia oleracea
  source 1..2223: /organism="Spinacia oleracea" /mol_type="unassigned DNA"
atgaacgatcgtaaagttatcgaactagagcaaggatgggagttcatggggaaggggattacgaagttgaaaaggattttggaaggattaccagagccgccttttaattcggaagactacatgatgctgtacacgacaatgtacaacatgtgtacacagaaaccccctcatgattactctcaacaactctatgacaattacaaagaggcatttgtggattacatacattcaacggttttaccttctttgggggacaaacatgatgagtttatgctgagagagcttgtgaagagatggtcaaatcataaagtaatggtgaggtggttgtctcgcttcttccattatctggatcggtacttcatcgctcggagatcgcttccttctttgaatgatgttggattgacgtgcttccgtgatctggtttatcaagaaatatctggcaaagccaaggatgctgttattgctctgattgatgaagaaagagagggtgggcaaattgacagagccttattgaagaatgtacttgatatatacgttgaaattggaatgacacaaatggattactacgaaaaggactttgaagctcatatgctggatgatactgctgcttattactcacgcaaggcctcaagctggattctggaggactcatgtccggaatacatgttgaagtcggaggagtgtttgaagaaagagaaagatagagtggctcattatctacattccagcagtgagccaaagcttctggagaaagtacaaaatgagttgctactggtttacgaaaatcagttgcttgagaaggagaattctggatgtcgtgcattgttgaaagatgacaaggtggaagatctttccaggatgtacaggctttatagcaaggttaccaaagggttggaacccattggcagtatcttcaaacagcatataaccgatgaaggaacagccctggtgcagcaggccgaagacgctgcaattagcaaggctgaaaatgctggcggtggttcacatgagcaggtcttcgtcaggaaagtgattgagttgcatgacaaatttatgacctatgttacagattgcttcaacagccataccatctttcacaaggctctcaaggaagcttttgaggtattcttaaacaagggtgttgctggtagttcaagtgctgaacttctagcttcattttgtgataatattctcaagaaaggtggtagtgaaaaattaagtgatgaggctattgaggattcactggagaaggtggtgaagcttctcgcatatgtcagtgataaagacctgtttgctgaattttacagaaagaagctctctcgccggctactctttgacaaaagtgctaatgatgatcatgagaggagtattttaacaaaattgaagcagcagtgtgggggacagttcacatcaaagatggaggggatggtgacagacttgacattggcgagggagaatcaaactaattttgaggaatatcttggacaaaatacagatgccagtcctggtcttgatttgactgtgacagttttgaccactgggttctggccaagttacaaatcttctgatcttaaccttcctgctgagatggtgaggtgtgttgaagtttttaagcaattttatcaaacaaagacaaaacacaggaagctcacctgggtatattcgttgggaagttgtaacattaatggcaagtttggtccgaaaacaattgaattggttgttggaacttatcaggctgctgcgctgatgctctttaacacatcagatcgactgagttattcagaaataacgacccaactaaatctagctgacgaagacttggttagagtgcttcaatctctatcttgcgcaaagtataagattcttctaaaagagccaagcacaagaaacgtgatctcaactgattgtttttcattcaactctaattttactgacagaatgaggaggattaggattcctcttcctccaatggatgagaggaaaaaggttgttgaagatgttgacaaagatagaagatatgctattgatgcctcaattgtacgcataatgaaaagtaggaaggctttgggatatcaacaattaatcacggagtgtgtggagcagctaagccgcatgttcaagcctgatttcaaagcaattaagaagaggatcgaggacttgataaccagagattatattgaaagagacaaggaaaaccctcagctattccggtacttggcttga

SEQ ID NO: 51 - DNA, 2220 bp, Beta vulgaris
  source 1..2220: /organism="Beta vulgaris" /mol_type="unassigned DNA"
atgaatgatcgtaaagttattgaactagagcaaggatgggagttcatggggaaggggattacaaagttgaagaggattctggaaggattgccagagccaccatttaattctgaagactacatgatgttgtacacgacgatgtacaatatgtgtactcagaaacccccacatgattactctcaacagctctatgacaattacaaacaggcttttgtggattacatcaactcgacggttttaccttctttgcgggagaagcatgatgagtttatgttaagagaacttgtgaaaagatgggcaaatcataaagtaatggtcaggtggttgtctcgtttcttccattatctggaccggtatttcattgctcggaggtcgcttccttctttgaatgaagttggactgacttgtttccgtgatctggtttatcaagaaatatctggcaaagccaaggatgctgttatagccctgattgatatagaaagagaaggtgggcagattgacagatcattattgaaaaatgtacttgatatatatgttgaaattggaatgggacaaatggatcactatgaaaaagactttgaagctcatatgctggatgatactgctgcttactactcgcgcaaagcgtctagctggattcttgaggactcttgtccggaatacatgttaaagtctgaggagtgtttgaagaaggagaaagagagagtggctaattatttacattccagcagtgagccaaagcttctggagaaagtgcaaaacgagttgctattggtttatgaaagccaattgcttgagaaggagaattcgggatgtcgtgcattactgaaagatgacaaggtggatgatctttccaggatgtacaggctttacagtaaggttaccaaaggattggaacccattggcagtatcttcaaacagcatataactgatgaaggaacagccttagtgcagcaggccgaagatgctgctatcagcaaggctgaaaatactggtggttcacatgagcaggtcttcgtcaggaaagtaatagagttgcatgacaaattcatgacttatgtcaccgattgcttcaacagccataccatatttcacaaggctcttaaggaggcttttgaggtatttttgaacaagggtgttgctggtagctcaagtgctgagttgctagctacattctgtgataacattctcaagaaaggtgggagcgaaaaactaagcgatgaggctattgaggattcacttgagaaggtggtgaagcttctggcctatgtcagtgataaagacctgtttgctgaattttacagaaagaagctctctcgccggctactctttgacaagagtgctaatgatgatcatgaaagaagtattttaaccaaattgaagcagcagtgtggcggacaattcacatcaaagatggaggggatggtgacagacttgaccttggcgagggagaatcaaactaattttgaggaatatcttagtcagaatccagatgccagtcctggtcttgatttgactgtgactgttctgacaactgggttctggccaagttacaaatcttccgatcttaaccttcccgctgagatggtgaggtgtgttgaagtttttaagcagttctattcaactaaaacaaagcacaggaagctgacctgggtttactcattgggaagctgtaatattaatggcaagtttggtccaaaaactattgaattggttgtcggaacttatcaggctgctgctttgatgctctttaacacatcagaccgactgagttattcagagatagcaactcaactaaatttagctgatgaagatctggttagagtgcttcaatctttatcctgcgcaaagtataagattcttttaaaggagccaaacacgaaaaccgtgtccccgactgattgtttttcatttaactctagtttcactgacaggatgaggaggataagaattcctcttcctccgatggatgagaggaaaaaggttgttgaggatgttgacaaagatagaagatatgctattgatgcctcaattgtacgcataatgaaaagtaggaaggttttggggtaccagcaattaatcacagagtgtgtggagcagctaagccgcatgttcaagcctgatttcaaggcaattaagaagaggatcgaggacttaataacccgagattatattgaaagagacaaggagaacccgcagctattccgatacttggcttga

SEQ ID NO: 52 - protein, 744 aa, Cucumis sativus
MTMGERKTIDLEQGWEFMQKGITKLKNILEGLPEPQFSSEDYMMLYTTMYNMCTQKPPHDYSQQLYDKYRESFEEYITSMVLPSLREKHDEFMLRELVKRWTNHKVMVRWLSRFFHYLDRYFIARRSLPPLNEVGLTCFRELVYKELNSKVRDAVISLIDQEREGEQIDRALLKNVLDIFVEIGMGQMDYYENDFEAAMLKDTAAYYSRKASNWILEDSCPDYMLKAEECLKREKDRVSHYLHSSSEPKLLEKVQHELLSVYATQLLEKEHSGCHALLRDDKVEDLSRMFRLFSKIPKGLDPVSNIFKQHVTAEGTALVKQAEDAASNKKAEKKDIVGLQEQVFVRKVIELHDKYLAYVNDCFQNHTLFHKALKEAFEVFCNKGVAGSSSAELLATFCDNILKKGGSEKLSDEAIEETLEKVVKLLAYICDKDLFAEFYRKKLARRLLFDKSANDDHERSILTKLKQQCGGQFTSKMEGMVTDLTLARENQTSFEEYLSNNPQASPGIDLTVTVLTTGFWPSYKSFDLNLPAEMVKCVEVFREFYQTKTKHRKLTWIYSLGTCNISGKFEPKTMELIVTTYQASALLLFNSSDRLSYSEIMTQLNLSDDDVVRLLHSLSCAKYKILNKEPNTKTISPNDHFEFNAKFSDKMRRIKIPLPPVDEKKKVIEDVDKDRRYAIDASIVRIMKSRKVLGHQQLVMECVEQLGRMFKPDFKAIKKRIEDLITRDYLERDKDNPHLFRYLA

SEQ ID NO: 53 - protein, 744 aa, Cucumis melo; identical to SEQ ID NO: 52

SEQ ID NO: 54 - protein, 744 aa, Cucurbita pepo
MTMGERKTIDLEQGWEFMQKGITKLKNILEGLPEPQFSSEDYMMLYTTMYNMCTQKPPHDYSQQLYDKYRESFEEYISSMVLPSLREKHDEFMLRELVKRWTNHKVMVRWLSRFFHYLDRYFIARRSLPPLNEVGLTCFRELVYKELNSKVRDAVISLIDQEREGEQIDRALLKNVLDIFVEIGMGQMDYYENDFEAAMLKDTAAYYSRKASNWILEDSCPDYMLKAEECLRREKDRVSHYLHSSSEPKLLEKVQHELLSVYATQLLEKEHSGCHALLRDDKVEDLSRMFRLFSKIPKGLDPVSNIFKQHVTAEGTALVKQAEDAASNKKAEKKDIVGLQEQVFVRKVIELHDKYLAYVNDCFQNHTLFHKALKEAFEVFCNKGVAGSSSAELLATFCDNILKKGGSEKLSDEAIEETLEKVVKLLAYICDKDLFAEFYRKKLARRLLFDKSANDDHERSILTKLKQQCGGQFTSKMEGMVTDLTLARENQTSFEEYLSNNPQASPGIDLTVTVLTTGFWPSYKSFDLNLPAEMVKCVEVFREFYQTKTKHRKLTWIYSLGTCNISGKFEPKTMELIVTTYQASALLLFNSSDKLSYSEIMTQLNLSDDDVVRLLHSLSCAKYKILNKEPNTKTISPNDHFEFNAKFSDKMRRIKIPLPPVDEKKKVIEDVDKDRRYAIDASIVRIMKSRKVLGHQQLVMECVEQLGRMFKPDFKAIKKRIEDLITRDYLERDKDNPHLFRYLA

SEQ ID NO: 55 - protein, 744 aa, citrillus lanatus; identical to SEQ ID NO: 52

SEQ ID NO: 56 - protein, 742 aa, Solanum melongena
MNQRSTIDLEHGWDFMQKGITKLKNILEGLPEPQFSSEDYMMLYTTMYNMCTQKPPHDYSQQLYDKYREAFEEYITTTVLPSLREKHDEFMLRELVKRWSNHKVMVRWLSRFFHYLDRYFIARRSLPGLNEVGLTCFRDLVYQELNGKVRDAVISLIDQEREGEQIDRALLKNVLDIFVEIGMGSMDYYENDFEAAMLKDTAAYYSRKASNWILEDSCPDYMLKAEECLKREKDRVSHYLHSSSETKLLEKVQHELLSVYANQLLEKEHSGCHALLRDDKVDDLSRMYRLFSKIPRGLEPVANIFKQHVTAEGTALVKQAEDAASNKKAEKRDVVGLQEQVFVRKVIELHDKYLAYVNNCFQNHTLFHKALKEAFELFCNKGVAGSSNAELLATFCDNILKKGGSEKLSDEAIEETLEKVVKLLAYISDKDLFAEFYRKKLARRLLFDKSANDEHERSILTKLKQQCGGQFTSKMEGMVTDLTLARENQASFEEYLSNNPTANPGIDLTVTVLTTGFWPSYKSFDLNLPAEMVRCVEVFKEFYQTKTKHRKLTWIYSLGTCNINGKFEAKTIELVVTTYQASALLLFNASDRLSYQEIMTQLNLSDDDVVRLLHSLSCAKYKILNKEPSTKTISPTDVFEFNSKFTDKMRRIKIPLPPVDEKKKVIEDVDKDRRYAIDASIVRIMKSRKVLGYQQLVMECVEQLGRMFKPDVKAIKKRIEDLITRDYLERDKDNPNLFKYLA

SEQ ID NO: 57 - protein, 742 aa, Solanum lycopersicum
MNQRSTIDLEHGWDFMQRGITKLKNILEGLPEPQFSSEDYMMLYTTMYNMCTQKPPHDYSQQLYDKYREAFEEYITTTVLPSLREKHDEFMLRELVKRWSNHKVMVRWLSRFFHYLDRYFIARRSLPGLNEVGLTCFRDQVYQELNGKVRDAVISLIDQEREGEQIDRALLKNVLDIFVEIGMGLMDYYENDFEAAMLKDTAAYYSRKASNWILEDSCPDYMLKAEECLKREKDRVSHYLHSSSETKLLEKVQHELLSVYATQLLEKEHSGCHALLRDDKVEDLSRMYRLFSKISRGLDPVANIFKQHVTAEGTALVKQAEDAASNKKAEKRDVVGLQEQVFVRKVIELHDKYLAYVNNCFQNHTLFHKALKEAFELFCNKGVAGSSSAELLATFCDNILKKGGSEKLSDEAIEETLEKVVKLLAYISDKDLFAEFYRKKLARRLLFDKSANDEHERSILTKLKQQCGGQFTSKMEGMVTDLTLARENQASFEEYLSNNPIANPGIDLTVTVLTTGFWPSYKSFDLNLPAEMVRCVEVFKEFYQTKTKHRKLTWIYSLGTCNINGKFEPKTIELVVTTYQASALLLFNASDRLSYQEIMTQLNLSDDDVVRLLHSLSCAKYKILNKEPSTKTISPTDVFEFNSKFTDKMRRIKIPLPPVDEKKKVIEDVDKDRRYAIDASIVRIMKSRKVLGYQQLVMECVEQLGRMFKPDVKAIKKRIEDLITRDYLERDKDNPNLFKYLA

SEQ ID NO: 58 - protein, 742 aa, Capsicum annuum
MNQRSTINLEHGWDFMQRGITKLKNILEGLPEPQFSSEDYMMLYTTMYNMCTQKPPHDYSQQLYDKYREAFEEYITTTVLPSLREKHDEFMLRELVKRWSNHKVMVRWLSRFFHYLDRYFIARRSLPGLNEVGLTCFRDLVYQELNGKVRDAVISLIDQEREGEQIDRALLKNVLDIFVEIGMGSMDYYENDFEAAMLKDTAAYYSRKASNWILEDSCPDYMLKAEECLKREKDRVSHYLHLSSETKLLEKVQHELLSVYATQLLEKEHSGCHALLRDDKVEDLSRMYRLFSKIPRGLDPVANIFKQHVTAEGTALVKQAEDAASNKKAEKRDVVGLQEQIFVRKVIELHDKYMAYVNNCFQNHTLFHKALKEAFELFCNKGVAGSSSAELLATFCDNILKKGGSEKLSDEAIEETLEKVVKLLAYISDKDLFAEFYRKKLARRLLFDKSANDEHERSILTKLKQQCGGQFTSKMEGMVTDLTLARENQASFEEYLSNNPAANPGIDLTVTVLTTGFWPSYKSFDLNLPAEMVRCVEVFKEFYQTKTKHRKLTWIYSLGTCNINGKFEPKTIELVVTTYQASALLLFNASDRLSYQEIMTQLNLSDDDVVRLLHSLSCAKYKILNKEPSTKTISPTDVFEFNFKFTDKMRRIKIPLPPVDEKKKVIEDVDKDRRYAIDASIVRIMKSRKVLGYQQLVMECVEQLGRMFKPDVKAIKKRIEDLITRDYLERDKDNPNLFKYLA

SEQ ID NO: 59 - protein, 738 aa, Brassica oleracea
MERKTIDLDQGWDYMQTGITKLKRILEGLPEPQFDSEQYMMLYTTMYNMCTQKPPHDYSQQLYDKYREAFEEYIHSTVLPALREKHDEYMLRELVKRWSNHKVMVRWLSRFFYYLDRYFIARRSLPPLNEVGLTCFRDLVYNELHSKVKDAVIALVDKEREGEQIDRALLKNVLDIYVEIGMGQMERYEEDFESFMLLDSASYYSRKASSWIQEDSCPDYMLKSEECLKKERERVAHYLHSSSEPKLVEKVQHELLVVYANQLLEKEHSGCRALLRDDKVDDLSRMYRLYHKIVKGLEPVANIFKQHVTAEGNALVQQAEDTATNHAANTASVQEQVLIRKVIELHDKYMVYVVECFQNHTLFHKALKEAFEIFCNKTVAGSSSAELLATFCDNILKKGGSEKLSDEAIEDTLEKVVKLLAYISDKDLFAEFYRKKLARRLLFDRSANDDHERSILTKLKQQCGGQFTSKMEGMVTDLTLARENQNSFEEYLGNNPAANPGIDLTVTVLTTGFWPSYKSFDINLPAEMVKCVEVFKGFYETKTKHRKLTWIYSLGTCHLNGKFDVKPIELVVSTYQAAVLLLFNTTDKLSYTDILTQLNLSHEDLVRLLHSLSCARYKILLKEPSTKTVSQSDSFEFNSKFTDRMRRIKIPLPPVDERKKVVEDVDKDRRYAIDAAIVRIMKSRKVLGHQQLVSECVEQLSRMFKPDIKAIKKRMEDLITRDYLERDKENANMFRYLA

SEQ ID NO: 60 - protein, 743 aa, Daucus carota
MMIERKTIDLEQGWDFMQKGITKLKNILEGFPEPQFSSEDYMMLYTTMYNMCTQKPPHDYSQQLYEKYREAIEEYITSTVLPSLREKHDEFMLRELVKRWSNHKVMVRWLSRFFHYLDRYFIARRSLPPLHEVGLTCFRDLVYQEINGKVRDAVISLINQEREGEQIDRALLKNVLDIFVEVGMSQMDYYENDFEADMLKDTAAYYSRKASNWILEDSCPDYMLKAEECLRREKDRVSNYLHSSSEPKLLEKVQHELLSHYATQLLEKEHSGCHALLRDDKVADLSRMYRLFSKIPRGLDPVSNIFKQHVTAEGTALVKQAEDAASNKKAEKRDVVGLQEQVFVRKIIELHDKYLTYVNDCFTNHTLFHKALKEAFEIFCNKGVSGSSSAELLATFCDNILKKGGSEKLSDEAIEETLEKVVRLLAYISDKDLFAEFYRKKLARRLLFDKSANDEHERSILTKLKQQCGGQFTSKMEGMVTDLTLAKENQSNFEEYLNNNSNVNPGIDLTVTVLTTGFWPSYKSFDLNLPAEMVKCVEVFREFYQTKTKHRKLTWIYSLGTCNIIGKFDPKTMELIVTTYQASALLLFNSSDRLSYNEIMTQLNLSDDDVVRLLHSLSCAKYKILSKEPNTKTISPTDCFQFNSKFTDKMRRIKIPLPPVDEKKKVIEDVDKDRRYAIDASIVRIMKSRKVLGYQQLVMECVEQLGRMFKPDVKAIKKRIEDLITRDYLERDKDNANLFRYLA

SEQ ID NO: 61 - protein, 742 aa, Apium graveolens
MNERKTIDLDNGWEFMQKGITKLKKILEGQPEPQFSSEDYMMLYTTMYNMCTQKPPHDYSQQLYDKYREAFEEYITSTVLPSLREKHDEFMLRELVNRWTNHKVMVRWLSRFFHYLDRYFIARRSLPALHEVGLTCFRDLVYQELKVKVRDAVISLIDQEREGEQIDRALLKNVLDIFVEIGMSQMDQYENDFEEAMLTDTAAYYSRKASNWILEDSCPDYMLKAEECLRREKDRVSHYLHFSSEPKLLEKVQHELLSVYATQLLEKEHSGCHALLRDDKVDDLSRMYRLFSKIPKGLDPVSYIFKQHVTNEGMALVKQAEDAASNKKAEKRDVVSLQEQVFVRKIIELHDKYLAYVNDCFTNHTLFHKALKEAFEIFCNKGVAGSSNAELLATFCDNILKKGGSEKLSDEAIEETLEKVVKLLAYISDKDLFAEFYRKKLARRLLFDKSANDEHERSILTKLKQQCGGQFTSKMEGMVTDLTLAKENQSSFEEYLGNNANVNPGIDLTVTVLTTGFWPSYKSFDLNLPAEMVKCVEVFREFYQTKTKHRKLTWIYSLGTCNINGKFEPKTIELIVTTYQASALLLFNTSDRLSYQEIMTQLNLSDDDVVRLLHSLSCAKYKILTKEPNNKTISPTDYFEFNSKFTDKMRRIKIPLPPVDEKKKVIEDVDKDRRYAIDASIVRIMKSRKVLGYQQLVMECVEQLGRMFKPDVKAIKKRIEDLITRDYLERDKDNANLFRYLA

SEQ ID NO: 62 - protein, 742 aa, Cichorium intybus
MNERKTIDLEQGWDFMQKGITKLKNILEGLPEPQFSSEDYMMLYTTMYNMCTQKPPHDYSQQLYDKYRESFEEYITSTVLPSLREKHDEFMLRELVRRWSNHKVMVRWLSRFFHYLDRYFIARRSLPPLNEVGLACFRDLVYQEVNGKVRDAVISLIDQEREGEQIDRALLKNVLDIFVEIGMGQMEYYENDFEASMLNDTAAYYSRKASNWILEDSCPDYMLKAEECLKREKDRVSHYLHSSSEPKLLEKVQTELLSVYATQLLEKEHSGCHALLRDDKVDDLSRMYRLFSKIQKGLDPVSSMFKQHVTAEGTTLVKQAEDAASTKKAEKRDVVGLQEQVFVRKVIELHDKYLAYVNDCFMNHTLFHKALKEAFEIFCNKGVAGSSSAELLATFCDNILKKGGSEKLSDEAIEDTLEKVVKLLAYISDKDLFAEFYRKKLARRLLFDKSANDEHERSILTKLKQQCGGQFTSKMEGMVTDLTLAKENQSHFEEYLNNNPNVSPGIDLTVTVLTTGFWPSYKSFDLNLPAEMVKCVEVFREFYQTKTKHRKLTWIYSLGTCNINGKFEPKTMELIVTTYQASALLLFNSSDRLSYQEIMTQLNLSDDDVVRLLHSLSCAKYKILLKEPNTKTISPTDFFEFNSKFTDKMRRIKIPLPPVDEKKKVIEDVDKDRRYAIDASIVRIMKSRKVLGYQQLVMECVEQLGRMFKPDVKAIKKRIEDLITRDYLERDKENPNLFRYLA

SEQ ID NO: 63 - protein, 742 aa, Cichorium endivia; identical to SEQ ID NO: 62

SEQ ID NO: 64 - protein, 744 aa, Allium ampeloprasum
MSLHERKTIDLEQGWAFMQKGITKLKNILDELNEPQFSSEDYMMLYTTMYNMCTQKPPHDYSQELYDKYRESFEEYITTTVLPSLREKHDEYMLRELVRRWSNHKIMVRWLSRFFHYLDRYFIARRSLPALNEVGLTCFRDLVYNEVHGKVKDAVISLIDQEREGEQIDRALLKNVLGIFVEIGLGSMECYENDFETSMLNATAAYYSRKASNWILEDSCPDYMLKAEECLKHEKDRVAHYLHSSSEQKLLEKVQHELLFVYASQLLEKEHSGCHALLRDDKVGDLSRMYRLFCRITRGLDPVSQIFKQHVTAEGTALVKHAEDAASNKKAEKKDIVGLQEQVFVRKVIELHDKYLAYVTDCFQNHSLFHKALKEAFEVFCNKGVAGSSSAELLAAFCDNILKKGGSEKLSDEAIEDTLEKVVKLLAYISDKDLFAEFYRKKLARRLLFDKSANDDHERSILTKLKQQCGGQFTSKMEGMVTDLTLARENQSSFDDYLSSNPKANSGIDLTVTVLTTGFWPSYKSFDLNLPDEMVKCVEIFKEFYETKTKHRKLTWIYSLGTCNINGKFETKTIELVVTTYQAAVLLLFNSADKLSYSEIVQQLNLSDDDVIRLLHSLSCAKYKILNKEPATKTITPNDHFEFNSKFTDRMRRIKIPLPPVDEKKKVIEDVDKDRRYAIDASIVRIMKSRKVLGHQQLVLECVEQLGRMFKPDFKAIKKRIEDLIARDYLERDKDNPNLFKYLA

SEQ ID NO: 65 - protein, 742 aa, Lactuca sativa
MNERKTIDLEQGWDFMQKGITKLKNILEGLPEPQFSSEDYMMLYTTMYNMCTQKPPHDYSQQLYDKYRESFEEYITSTVLPSLREKHDEFMLRELVRRWSNHKVMVRWLSRFFHYLDRYFIARRSLPPLNEVGLACFRDLVYQEVNGKVRDAVISLIDQEREGEQIDRALLKNVLDIFVEIGMGQMEYYENDFEASMLNDTAAYYSRKASNWILEDSCPDYMLKAEECLKREKDRVSHYLHSSSEPKLLEKVQNELLSVYATQLLEKEHSGCHALLRDDKVDDLSRMYRLFSKIPKGLDPVSSMFKQHVTAEGTTLVKQAEDAASTKKAEKRDVVGLQEQVFVRKVIELHDKYLAYVNDCFMNHTLFHKALKEAFEIFCNKGVAGSSSAELLATFCDNILKKGGSEKLSDEAIEDTLEKVVKLLAYISDKDLFAEFYRKKLARRLLFDKSANDEHERSILTKLKQQCGGQFTSKMEGMVTDLTLAKENQSHFEEYLNNNPNVSPGIDLTVTVLTTGFWPSYKSFDLNLPAEMVKCVEVFREFYQTKTKHRKLTWIYSLGTCNINGKFEPKTMELIVTTYQASALLLFNLSDRLSYQEIMTQLNLSDDDVVRLLHSLSCAKYKILLKEPNTKTISPTDYFEFNSKFTDKMRRIKIPLPPVDEKKKVIEDVDKDRRYAIDASIVRIMKSRKVLGYQQLVMECVEQLGRMFKPDVKAIKKRIEDLITRDYLERDKENPNLFRYLA

SEQ ID NO: 66 - protein, 738 aa, Raphanus sativus
MERKTIDLEQGWDYMQTGITKLKRILEGLPEPQFDSEQYMMLYTTMYNMCTQKPPHDYSQQLYDKYREAFEEYIDSTVLPALKEKHDEYMLRELVKRWSNHKVMVRWLSRFFYYLDRYFIARRSLPPLNEVGLTCFRDRVYKELHSKVKDAVIALVDKEREGEQIDRALLKNVLDIYVEIGMGQMERYEVDFESFMLLDSASYYSRKASNWIQEDSCPDYMLKSEECLKKERERVAHYLHSSSEPKLVEKVQHELLVVYANQLLEKEHSGCRALLRDDKVDDLSRMYRLYHKIAKGLEPVANIFKQHVTAEGNALVQQAEDTATNQAANTASVQEQVLIRKVIELHDKYMVYVVECFQNHTLFHKALKEAFEIFCNKTVAGSSSAELLATFCDNILKKGGSEKLSDEAIEDTLEKVVKLLAYISDKDLFAEFYRKKLARRLLFDRSANDDHERSILTKLKQQCGGQFTSKMEGMVTDLTLARENQTSFEEYLGNNPAANPGIDLTVTVLTTGFWPSYKSFDINLPSEMVKCVEVFKGFYETKTKHRKLTWIYSLGTCHLNGKFDHKPIELVVSTYQAAVLLLFNTTDKLSYNDILTQLNLSHEDLVRLLHSLSCARYKILLKEPSTKTVTQTDSFEFNAKFTDRMRRIKIPLPPVDERKKVVEDVDKDRRYAIDAAIVRIMKSRKVLGHQQLVSECVEQLSRMFKPDIKAIKKRMEDLITRDYLERDKENPNMFRYLA

SEQ ID NO: 67 - protein, 740 aa, Spinacia oleracea
MNDRKVIELEQGWEFMGKGITKLKRILEGLPEPPFNSEDYMMLYTTMYNMCTQKPPHDYSQQLYDNYKEAFVDYIHSTVLPSLGDKHDEFMLRELVKRWSNHKVMVRWLSRFFHYLDRYFIARRSLPSLNDVGLTCFRDLVYQEISGKAKDAVIALIDEEREGGQIDRALLKNVLDIYVEIGMTQMDYYEKDFEAHMLDDTAAYYSRKASSWILEDSCPEYMLKSEECLKKEKDRVAHYLHSSSEPKLLEKVQNELLLVYENQLLEKENSGCRALLKDDKVEDLSRMYRLYSKVTKGLEPIGSIFKQHITDEGTALVQQAEDAAISKAENAGGGSHEQVFVRKVIELHDKFMTYVTDCFNSHTIFHKALKEAFEVFLNKGVAGSSSAELLASFCDNILKKGGSEKLSDEAIEDSLEKVVKLLAYVSDKDLFAEFYRKKLSRRLLFDKSANDDHERSILTKLKQQCGGQFTSKMEGMVTDLTLARENQTNFEEYLGQNTDASPGLDLTVTVLTTGFWPSYKSSDLNLPAEMVRCVEVFKQFYQTKTKHRKLTWVYSLGSCNINGKFGPKTIELVVGTYQAAALMLFNTSDRLSYSEITTQLNLADEDLVRVLQSLSCAKYKILLKEPSTRNVISTDCFSFNSNFTDRMRRIRIPLPPMDERKKVVEDVDKDRRYAIDASIVRIMKSRKALGYQQLITECVEQLSRMFKPDFKAIKKRIEDLITRDYIERDKENPQLFRYLA

SEQ ID NO: 68 - protein, 739 aa, Beta vulgaris
MNDRKVIELEQGWEFMGKGITKLKRILEGLPEPPFNSEDYMMLYTTMYNMCTQKPPHDYSQQLYDNYKQAFVDYINSTVLPSLREKHDEFMLRELVKRWANHKVMVRWLSRFFHYLDRYFIARRSLPSLNEVGLTCFRDLVYQEISGKAKDAVIALIDIEREGGQIDRSLLKNVLDIYVEIGMGQMDHYEKDFEAHMLDDTAAYYSRKASSWILEDSCPEYMLKSEECLKKEKERVANYLHSSSEPKLLEKVQNELLLVYESQLLEKENSGCRALLKDDKVDDLSRMYRLYSKVTKGLEPIGSIFKQHITDEGTALVQQAEDAAISKAENTGGSHEQVFVRKVIELHDKFMTYVTDCFNSHTIFHKALKEAFEVFLNKGVAGSSSAELLATFCDNILKKGGSEKLSDEAIEDSLEKVVKLLAYVSDKDLFAEFYRKKLSRRLLFDKSANDDHERSILTKLKQQCGGQFTSKMEGMVTDLTLARENQTNFEEYLSQNPDASPGLDLTVTVLTTGFWPSYKSSDLNLPAEMVRCVEVFKQFYSTKTKHRKLTWVYSLGSCNINGKFGPKTIELVVGTYQAAALMLFNTSDRLSYSEIATQLNLADEDLVRVLQSLSCAKYKILLKEPNTKTVSPTDCFSFNSSFTDRMRRIRIPLPPMDERKKVVEDVDKDRRYAIDASIVRIMKSRKVLGYQQLITECVEQLSRMFKPDFKAIKKRIEDLITRDYIERDKENPQLFRYLA

SEQ ID NO: 69 - protein, 738 aa, Arabidopsis
MERKTIDLEQGWDYMQTGITKLKRILEGLNEPAFDSEQYMMLYTTIYNMCTQKPPHDYSQQLYDKYREAFEEYINSTVLPALREKHDEFMLRELFKRWSNHKVMVRWLSRFFYYLDRYFIARRSLPPLNEVGLTCFRDLVYNELHSKVKQAVIALVDKEREGEQIDRALLKNVLDIYVEIGMGQMERYEEDFESFMLQDTSSYYSRKASSWIQEDSCPDYMLKSEECLKKERERVAHYLHSSSEPKLVEKVQHELLVVFASQLLEKEHSGCRALLRDDKVDDLSRMYRLYHKILRGLEPVANIFKQHVTAEGNALVQQAEDTATNQVANTASVQEQVLIRKVIELHDKYMVYVTECFQNHTLFHKALKEAFEIFCNKTVAGSSSAELLATFCDNILKKGGSEKLSDEAIEDTLEKVVKLLAYISDKDLFAEFYRKKLARRLLFDRSANDDHERSILTKLKQQCGGQFTSKMEGMVTDLTLARENQNSFEDYLGSNPAANPGIDLTVTVLTTGFWPSYKSFDINLPSEMIKCVEVFKGFYETKTKHRKLTWIYSLGTCHINGKFDQKAIELIVSTYQAAVLLLFNTTDKLSYTEILAQLNLSHEDLVRLLHSLSCAKYKILLKEPNTKTVSQNDAFEFNSKFTDRMRRIKIPLPPVDERKKVVEDVDKDRRYAIDAAIVRIMKSRKVLGHQQLVSECVEQLSRMFKPDIKAIKKRMEDLITRDYLERDKENPNMFRYLA